European Patent Specification EP 3 981 419 B1, published June 24, 2026. Title: BioUltraBond - a novel sealant, glue or filler for biological tissues. Applicant: Albert-Ludwigs-Universität Freiburg. The sequence listing filed with the application follows.

SEQUENCE LISTING (117 sequences)

SEQ ID NO: 1 - protein, 102 aa, Homo sapiens
  N-terminal domain of human SATB1
GTMLPVFCVVEHYENAIEYDCKEEHAEFVLVRKDMLFNQLIEMALLSLGYSHSSAAQAKGLIQVGKWNPVPLSYVTDAPDATVADMLQDVYHVVTLKIQLHS

SEQ ID NO: 2 - protein, 102 aa, Canis lupus familiaris; identical to SEQ ID NO: 1
  dog, Canis lupus familiaris, DNA-binding protein SATB1, NCBI Reference XP_022264105.1, N-terminal sequence

SEQ ID NO: 3 - protein, 102 aa, Canis lupus familiaris
  dog, Canis lupus familiaris, DNA-binding protein SATB2 isoform X1, NCBI Reference Sequence: XP_005640560.1, N-terminal domain;
GLMIPVFCVVEQLDGSLEYDNREEHAEFVLVRKDVLFSQLVETALLALGYSHSSAAQAQGIIKLGRWNPLPLSYVTDAPDATVADMLQDVYHVVTLKIQLQS

SEQ ID NO: 4 - protein, 102 aa, Felis catus; identical to SEQ ID NO: 1
  cat, Felis catus, DNA-binding protein SATB1 isoform X4, NCBI Reference XP_011284516.1, N-terminal sequence,

SEQ ID NO: 5 - protein, 102 aa, Equus caballus; identical to SEQ ID NO: 1
  horse, Equus caballus, DNA-binding protein SATB1 isoform X1, NCBI Reference: XP_014587330.2, N-terminal sequence,

SEQ ID NO: 6 - protein, 102 aa, Sus scrofa; identical to SEQ ID NO: 1
  pig, Sus scrofa, DNA-binding protein SATB1, NCBI Reference: XP_003358373.2, N-terminal sequence,

SEQ ID NO: 7 - protein, 102 aa, Sus scrofa; identical to SEQ ID NO: 3
  pig, Sus scrofa, DNA-binding protein SATB2 isoform X1, NCBI Reference: XP_020931727.1, N-terminal sequence,

SEQ ID NO: 8 - protein, 102 aa, Bos taurus; identical to SEQ ID NO: 1
  cow, Bos taurus, DNA-binding protein SATB1, NCBI Reference: NP_001095510.1, N-terminal sequence,

SEQ ID NO: 9 - protein, 102 aa, Bos taurus; identical to SEQ ID NO: 3
  cow, Bos taurus, DNA-binding protein SATB2, NCBI Reference: NP001192999.1, N-terminal sequence,

SEQ ID NO: 10 - protein, 102 aa, Ovis aries; identical to SEQ ID NO: 1
  sheep, Ovis aries, DNA-binding protein SATB1, NCBI-reference: XP_027817855.1, N-terminal sequence,

SEQ ID NO: 11 - protein, 102 aa, Cavia porcellus; identical to SEQ ID NO: 1
  Guinea pig, Cavia porcellus, DNA-binding protein SATB1 isoform X1, NCBI Reference: XP_005008358.1, N-terminal sequence,

SEQ ID NO: 12 - protein, 102 aa, Oryctolagus cuniculus; identical to SEQ ID NO: 1
  rabbit (Oryctolagus cuniculus, DNA-binding protein SATB1, NCBI-reference: XP_008264272.1, N-terminal sequence,

SEQ ID NO: 13 - protein, 102 aa, Microtus ochrogaster; identical to SEQ ID NO: 1
  rodent, prairie vole, Microtus ochrogaster, DNA-binding protein SATB1 isoform X1, NCBI-reference: XP_005368803.1, N-terminal sequence,

SEQ ID NO: 14 - protein, 102 aa, Gallus gallus
  Chicken, Gallus gallus, DNA-binding protein SATB1, NCBI Reference: NP_001186573.1, N-terminal sequence,
GSMLPVFCVVEHYENAIEYDSKEEHAEFVLVRKDMLFNQLIEMALLSLGYSHSSAAQAKGLIQVGKWNPVPLSYVTDAPDATVADMLQDVYHVVTLKIQLHS

SEQ ID NO: 15 - protein, 102 aa, Alligator mississippiensis; identical to SEQ ID NO: 14
  Alligator, (amphibian) Alligator mississippiensis, DNA-binding protein SATB2, NCBI Reference: KYO26889.1, N-terminal sequence

SEQ ID NO: 16 - protein, 102 aa, Oncorhynchus kisutch
  Fish, Oncorhynchus kisutch engl. coho salmon, deutsch Silberlachs, DNA-binding protein SATB1-like isoform X1, NCBI Reference: XP_031642577.1, N-terminal sequence,
GNMLPVFCVVEHYESPIEFDSKEEHAEFVLVRKDMLFNQLIEMALLSLGYSHSSAAQAKGLIQVGKWNPVPLSYVTDAPDATVADMLQDVYHVVTLKIQLHS

SEQ ID NO: 17 - protein, 102 aa, Oncorhynchus mykiss; identical to SEQ ID NO: 16
  Fish, Oncorhynchus mykiss, eng. rainbow trout, dt. Regenbogenforelle, DNA-binding protein SATB1-like isoform X6, NCBI Reference: XP_021450053.1, N-terminal sequence

SEQ ID NO: 18 - protein, 102 aa, Oncorhynchus mykiss
  Fish, Oncorhynchus mykiss, DNA-binding protein SATB1-like, NCBI Reference: XP_021417777.1, N-terminal sequence
LPVLCVVEHRENPVSAVEAERREEHAEFVLVRRDLLFNQLIEMALLALGYSHSSAAQAKGLIQVGRWNPVPLSCVTDAPDATVADMLQDLYHVTTLKIQLTR

SEQ ID NO: 19 - DNA, 711 bp, Streptococcus pyogenes
ggtcaggacggtcgtaacggtgaacgtggtgaacagggtccgaccggtccgaccggtccggctggtccgcgtggtctgcagggtctgcagggtctgcagggtgaacgtggtgaacagggtccgaccggtccggctggtccgcgtggtctgcagggtgaacgtggtgaacagggtccgaccggtctggctggtaaagctggtgaagctggtgctaaaggtgaaaccggtccggctggtccgcagggtccgcgtggtgaacagggtccgcagggtctgccgggtaaagacggtgaagctggtgctcagggtccggctggtccgatgggtccggctggtgaacgtggtgaaaaaggtgaaccgggtacccagggtgctaaaggtgaccgtggtgaaaccggtccggttggtccgcgtggtgaacgtggtgaagctggtccggctggtaaagacggtgaacgtggtccggttggtccggctggtaaagacggtcagaacggtcaggacggtctgccgggtaaagacggtaaagacggtcagaacggtaaagacggtctgccgggtaaagacggtaaagacggtcagaacggtaaagacggtctgccgggtaaagacggtaaagacggtcaggacggtaaagacggtctgccgggtaaagacggtaaagacggtctgccgggtaaagacggtaaagacggtcagccgggtaaaccg

SEQ ID NO: 20 - protein, 237 aa, Streptococcus pyogenes
  Bacterial collagene-like protein: Scl2.28CL (from protein P163, collagen-like region with 79 Gly-Xaa-Yaa/GXY repeats, from (1) derived from Streptococcus pyogenes Scl2 protein, GenBank: AY069936.1)
GQDGRNGERGEQGPTGPTGPAGPRGLQGLQGLQGERGEQGPTGPAGPRGLQGERGEQGPTGLAGKAGEAGAKGETGPAGPQGPRGEQGPQGLPGKDGEAGAQGPAGPMGPAGERGEKGEPGTQGAKGDRGETGPVGPRGERGEAGPAGKDGERGPVGPAGKDGQNGQDGLPGKDGKDGQNGKDGLPGKDGKDGQNGKDGLPGKDGKDGQDGKDGLPGKDGKDGLPGKDGKDGQPGKP

SEQ ID NO: 21 - DNA, 3207 bp, Homo sapiens
  /note="COL1A1 human: UniProtKB - Q6LAN8 (Q6LAN8_HUMAN: Collagen type I alpha 1)" /note="COL1A1 human: UniProtKB - Q6LAN8 (Q6LAN8_HUMAN: Collagen type I alpha 1), aa 1-22 signal peptide; aa 23 - 1069 col1A1 chain"
atgttcagctttgtggacctccggctcctgctcctcttagcggccaccgccctcctgacgcacggccaagaggaaggccaagtcgagggccaagacgaagacatcccaccaatcacctgcgtacagaacggcctcaggtaccatgaccgagacgtgtggaaacccgagccctgccggatctgcgtctgcgacaacggcaaggtgttgtgcgatgacgtgatctgtgacgagaccaagaactgccccggcgccgaagtccccgagggcgagtgctgtcccgtctgccccgacggctcagagtcacccaccgaccaagaaaccaccggcgtcgagggacccaagggagacactggcccccgaggcccaaggggacccgcaggcccccctggccgagatggcatccctggacagcctggacttcccggaccccccggaccccccggacctcccggaccccctggcctcggaggaaactttgctccccagctgtcttatggctatgatgagaaatcaaccggaggaatttccgtgcctggccccatgggtccctctggtcctcgtggtctccctggcccccctggtgcacctggtccccaaggcttccaaggtccccctggtgagcctggcgagcctggagcttcaggtcccatgggtccccgaggtcccccaggtccccctggaaagaatggagatgatggggaagctggaaaacctggtcgtcctggtgagcgtgggcctcctgggcctcagggtgctcgaggattgcccggaacagctggcctccctggaatgaagggacacagaggtttcagtggtttggatggtgccaagggagatgctggtcctgctggtcctaagggtgagcctggcagccctggtgaaaatggagctcctggtcagatgggcccccgtggcctgcctggtgagagaggtcgccctggagcccctggccctgctggtgctcgtggaaatgatggtgctactggtgctgccgggccccctggtcccaccggccccgctggtcctcctggcttccctggtgctgttggtgctaagggtgaagctggtccccaagggccccgaggctctgaaggtccccagggtgtgcgtggtgagcctggcccccctggccctgctggtgctgctggccctgctggaaaccctggtgctgatggacagcctggtgctaaaggtgccaatggtgctcctggtattgctggtgctcctggcttccctggtgcccgaggcccctctggaccccagggccccggcggccctcctggtcccaagggtaacagcggtgaacctggtgctcctggcagcaaaggagacactggtgctaagggagagcctggccctgttggtgttcaaggaccccctggccctgctggagaggaaggaaagcgaggagctcgaggtgaacccggacccactggcctgcccggaccccctggcgagcgtggtggacctggtagccgtggtttccctggcgcagatggtgttgctggtcccaagggtcccgctggtgaacgtggttctcctggccctgctggccccaaaggatctcctggtgaagctggtcgtcccggtgaagctggtctgcctggtgccaagggtctgactggaagccctggcagccctggtcctgatggcaaaactggcccccctggtcccgccggtcaagatggtcgccccggacccccaggcccacctggtgcccgtggtcaggctggtgtgatgggattccctggacctaaaggtgctgctggagagcccggcaaggctggagagcgaggtgttcccggaccccctggcgctgtcggtcctgctggcaaagatggagaggctggagctcagggaccccctggccctgctggtcccgctggcgagagaggtgaacaaggccctgctggctcccccggattccagggtctccctggtcctgctggtcctccaggtgaagcaggcaaacctggtgaacagggtgttcctggagaccttggcgcccctggcccctctggagcaagaggcgagagaggtttccctggcgagcgtggtgtgcaaggtccccctggtcctgctggtccccgaggggccaacggtgctcccggcaacgatggtgctaagggtgatgctggtgcccctggagctcccggtagccagggcgcccctggccttcagggaatgcctggtgaacgtggtgcagctggtcttccagggcctaagggtgacagaggtgatgctggtcccaaaggtgctgatggctctcctggcaaagatggcgtccgtggtctgaccggccccattggtcctcctggccctgctggtgcccctggtgacaagggtgaaagtggtcccagcggccctgctggtcccactggagctcgtggtgcccccggagaccgtggtgagcctggtccccccggccctgctggctttgctggcccccctggtgctgacggccaacctggtgctaaaggcgaacctggtgatgctggtgctaaaggcgatgctggtccccctggccctgccggacccgctggaccccctggccccattggtaatgttggtgctcctggagccaaaggtgctcgcggcagcgctggtccccctggtgctactggtttccctggtgctgctggccgagtcggtcctcctggcccctctggaaatgctggaccccctggccctcctggtcctgctggcaaagaaggcggcaaaggtccccgtggtgagactggccctgctggacgtcctggtgaagttggtccccctggtccccctggccctgctggcgagaaaggatcccctggtgctgatggtcctgctggtgctcctggtactcccgggcctcaaggtattgctggacagcgtggtgtggtcggcctgcctggtcagagaggagagagaggcttccctggtcttcctggcccctctggtgaacctggcaaacaaggtccctctggagcaagtggtgaacgtggtccccctggtcccatgggcccccctggattggctggaccccctggtgaatctggacgtgagggggctcctggtgccgaaggttcccctggacgagacggttctcctggcgccaagggtgaccgtggtgagaccggccccgctggaccccctggtgctcctggtgctcctggtgcccctggccccgttggccctgctggcaagagtggtgatcgtggtgagact

SEQ ID NO: 22 - protein, 3207 aa, Homo sapiens
  COL1A1 human: UniProtKB - Q6LAN8 (Q6LAN8_HUMAN: Collagen type I alpha 1)
ATGTTCAGCTTTGTGGACCTCCGGCTCCTGCTCCTCTTAGCGGCCACCGCCCTCCTGACGCACGGCCAAGAGGAAGGCCAAGTCGAGGGCCAAGACGAAGACATCCCACCAATCACCTGCGTACAGAACGGCCTCAGGTACCATGACCGAGACGTGTGGAAACCCGAGCCCTGCCGGATCTGCGTCTGCGACAACGGCAAGGTGTTGTGCGATGACGTGATCTGTGACGAGACCAAGAACTGCCCCGGCGCCGAAGTCCCCGAGGGCGAGTGCTGTCCCGTCTGCCCCGACGGCTCAGAGTCACCCACCGACCAAGAAACCACCGGCGTCGAGGGACCCAAGGGAGACACTGGCCCCCGAGGCCCAAGGGGACCCGCAGGCCCCCCTGGCCGAGATGGCATCCCTGGACAGCCTGGACTTCCCGGACCCCCCGGACCCCCCGGACCTCCCGGACCCCCTGGCCTCGGAGGAAACTTTGCTCCCCAGCTGTCTTATGGCTATGATGAGAAATCAACCGGAGGAATTTCCGTGCCTGGCCCCATGGGTCCCTCTGGTCCTCGTGGTCTCCCTGGCCCCCCTGGTGCACCTGGTCCCCAAGGCTTCCAAGGTCCCCCTGGTGAGCCTGGCGAGCCTGGAGCTTCAGGTCCCATGGGTCCCCGAGGTCCCCCAGGTCCCCCTGGAAAGAATGGAGATGATGGGGAAGCTGGAAAACCTGGTCGTCCTGGTGAGCGTGGGCCTCCTGGGCCTCAGGGTGCTCGAGGATTGCCCGGAACAGCTGGCCTCCCTGGAATGAAGGGACACAGAGGTTTCAGTGGTTTGGATGGTGCCAAGGGAGATGCTGGTCCTGCTGGTCCTAAGGGTGAGCCTGGCAGCCCTGGTGAAAATGGAGCTCCTGGTCAGATGGGCCCCCGTGGCCTGCCTGGTGAGAGAGGTCGCCCTGGAGCCCCTGGCCCTGCTGGTGCTCGTGGAAATGATGGTGCTACTGGTGCTGCCGGGCCCCCTGGTCCCACCGGCCCCGCTGGTCCTCCTGGCTTCCCTGGTGCTGTTGGTGCTAAGGGTGAAGCTGGTCCCCAAGGGCCCCGAGGCTCTGAAGGTCCCCAGGGTGTGCGTGGTGAGCCTGGCCCCCCTGGCCCTGCTGGTGCTGCTGGCCCTGCTGGAAACCCTGGTGCTGATGGACAGCCTGGTGCTAAAGGTGCCAATGGTGCTCCTGGTATTGCTGGTGCTCCTGGCTTCCCTGGTGCCCGAGGCCCCTCTGGACCCCAGGGCCCCGGCGGCCCTCCTGGTCCCAAGGGTAACAGCGGTGAACCTGGTGCTCCTGGCAGCAAAGGAGACACTGGTGCTAAGGGAGAGCCTGGCCCTGTTGGTGTTCAAGGACCCCCTGGCCCTGCTGGAGAGGAAGGAAAGCGAGGAGCTCGAGGTGAACCCGGACCCACTGGCCTGCCCGGACCCCCTGGCGAGCGTGGTGGACCTGGTAGCCGTGGTTTCCCTGGCGCAGATGGTGTTGCTGGTCCCAAGGGTCCCGCTGGTGAACGTGGTTCTCCTGGCCCTGCTGGCCCCAAAGGATCTCCTGGTGAAGCTGGTCGTCCCGGTGAAGCTGGTCTGCCTGGTGCCAAGGGTCTGACTGGAAGCCCTGGCAGCCCTGGTCCTGATGGCAAAACTGGCCCCCCTGGTCCCGCCGGTCAAGATGGTCGCCCCGGACCCCCAGGCCCACCTGGTGCCCGTGGTCAGGCTGGTGTGATGGGATTCCCTGGACCTAAAGGTGCTGCTGGAGAGCCCGGCAAGGCTGGAGAGCGAGGTGTTCCCGGACCCCCTGGCGCTGTCGGTCCTGCTGGCAAAGATGGAGAGGCTGGAGCTCAGGGACCCCCTGGCCCTGCTGGTCCCGCTGGCGAGAGAGGTGAACAAGGCCCTGCTGGCTCCCCCGGATTCCAGGGTCTCCCTGGTCCTGCTGGTCCTCCAGGTGAAGCAGGCAAACCTGGTGAACAGGGTGTTCCTGGAGACCTTGGCGCCCCTGGCCCCTCTGGAGCAAGAGGCGAGAGAGGTTTCCCTGGCGAGCGTGGTGTGCAAGGTCCCCCTGGTCCTGCTGGTCCCCGAGGGGCCAACGGTGCTCCCGGCAACGATGGTGCTAAGGGTGATGCTGGTGCCCCTGGAGCTCCCGGTAGCCAGGGCGCCCCTGGCCTTCAGGGAATGCCTGGTGAACGTGGTGCAGCTGGTCTTCCAGGGCCTAAGGGTGACAGAGGTGATGCTGGTCCCAAAGGTGCTGATGGCTCTCCTGGCAAAGATGGCGTCCGTGGTCTGACCGGCCCCATTGGTCCTCCTGGCCCTGCTGGTGCCCCTGGTGACAAGGGTGAAAGTGGTCCCAGCGGCCCTGCTGGTCCCACTGGAGCTCGTGGTGCCCCCGGAGACCGTGGTGAGCCTGGTCCCCCCGGCCCTGCTGGCTTTGCTGGCCCCCCTGGTGCTGACGGCCAACCTGGTGCTAAAGGCGAACCTGGTGATGCTGGTGCTAAAGGCGATGCTGGTCCCCCTGGCCCTGCCGGACCCGCTGGACCCCCTGGCCCCATTGGTAATGTTGGTGCTCCTGGAGCCAAAGGTGCTCGCGGCAGCGCTGGTCCCCCTGGTGCTACTGGTTTCCCTGGTGCTGCTGGCCGAGTCGGTCCTCCTGGCCCCTCTGGAAATGCTGGACCCCCTGGCCCTCCTGGTCCTGCTGGCAAAGAAGGCGGCAAAGGTCCCCGTGGTGAGACTGGCCCTGCTGGACGTCCTGGTGAAGTTGGTCCCCCTGGTCCCCCTGGCCCTGCTGGCGAGAAAGGATCCCCTGGTGCTGATGGTCCTGCTGGTGCTCCTGGTACTCCCGGGCCTCAAGGTATTGCTGGACAGCGTGGTGTGGTCGGCCTGCCTGGTCAGAGAGGAGAGAGAGGCTTCCCTGGTCTTCCTGGCCCCTCTGGTGAACCTGGCAAACAAGGTCCCTCTGGAGCAAGTGGTGAACGTGGTCCCCCTGGTCCCATGGGCCCCCCTGGATTGGCTGGACCCCCTGGTGAATCTGGACGTGAGGGGGCTCCTGGTGCCGAAGGTTCCCCTGGACGAGACGGTTCTCCTGGCGCCAAGGGTGACCGTGGTGAGACCGGCCCCGCTGGACCCCCTGGTGCTCCTGGTGCTCCTGGTGCCCCTGGCCCCGTTGGCCCTGCTGGCAAGAGTGGTGATCGTGGTGAGACT

SEQ ID NO: 23 - DNA, 2358 bp, Homo sapiens
  Elastin (human): UniProtKB - P15502 (ELN_HUMAN); aa 1 - 26 signal peptide; aa 27 - 786 elastin chain
atggccggcctgaccgccgccgccccccgccccggcgtgctgctgctgctgctgagcatcctgcaccccagccgccccggcggcgtgcccggcgccatccccggcggcgtgcccggcggcgtgttctaccccggcgccggcctgggcgccctgggcggcggcgccctgggccccggcggcaagcccctgaagcccgtgcccggcggcctggccggcgccggcctgggcgccggcctgggcgccttccccgccgtgaccttccccggcgccctggtgcccggcggcgtggccgacgccgccgccgcctacaaggccgccaaggccggcgccggcctgggcggcgtgcccggcgtgggcggcctgggcgtgagcgccggcgccgtggtgccccagcccggcgccggcgtgaagcccggcaaggtgcccggcgtgggcctgcccggcgtgtaccccggcggcgtgctgcccggcgcccgcttccccggcgtgggcgtgctgcccggcgtgcccaccggcgccggcgtgaagcccaaggcccccggcgtgggcggcgccttcgccggcatccccggcgtgggccccttcggcggcccccagcccggcgtgcccctgggctaccccatcaaggcccccaagctgcccggcggctacggcctgccctacaccaccggcaagctgccctacggctacggccccggcggcgtggccggcgccgccggcaaggccggctaccccaccggcaccggcgtgggcccccaggccgccgccgccgccgccgccaaggccgccgccaagttcggcgccggcgccgccggcgtgctgcccggcgtgggcggcgccggcgtgcccggcgtgcccggcgccatccccggcatcggcggcatcgccggcgtgggcacccccgccgccgccgccgccgccgccgccgccgccaaggccgccaagtacggcgccgccgccggcctggtgcccggcggccccggcttcggccccggcgtggtgggcgtgcccggcgccggcgtgcccggcgtgggcgtgcccggcgccggcatccccgtggtgcccggcgccggcatccccggcgccgccgtgcccggcgtggtgagccccgaggccgccgccaaggccgccgccaaggccgccaagtacggcgcccgccccggcgtgggcgtgggcggcatccccacctacggcgtgggcgccggcggcttccccggcttcggcgtgggcgtgggcggcatccccggcgtggccggcgtgcccggcgtgggcggcgtgcccggcgtgggcggcgtgcccggcgtgggcatcagccccgaggcccaggccgccgccgccgccaaggccgccaagtacggcgccgccggcgccggcgtgctgggcggcctggtgcccggcgcccccggcgccgtgcccggcgtgcccggcaccggcggcgtgcccggcgtgggcacccccgccgccgccgccgccaaggccgccgccaaggccgcccagttcggcctggtgcccggcgtgggcgtggcccccggcgtgggcgtggcccccggcgtgggcgtggcccccggcgtgggcctggcccccggcgtgggcgtggcccccggcgtgggcgtggcccccggcgtgggcgtggcccccggcatcggccccggcggcgtggccgccgccgccaagagcgccgccaaggtggccgccaaggcccagctgcgcgccgccgccggcctgggcgccggcatccccggcctgggcgtgggcgtgggcgtgcccggcctgggcgtgggcgccggcgtgcccggcctgggcgtgggcgccggcgtgcccggcttcggcgccggcgccgacgagggcgtgcgccgcagcctgagccccgagctgcgcgagggcgaccccagcagcagccagcacctgcccagcacccccagcagcccccgcgtgcccggcgccctggccgccgccaaggccgccaagtacggcgccgccgtgcccggcgtgctgggcggcctgggcgccctgggcggcgtgggcatccccggcggcgtggtgggcgccggccccgccgccgccgccgccgccgccaaggccgccgccaaggccgcccagttcggcctggtgggcgccgccggcctgggcggcctgggcgtgggcggcctgggcgtgcccggcgtgggcggcctgggcggcatcccccccgccgccgccgccaaggccgccaagtacggcgccgccggcctgggcggcgtgctgggcggcgccggccagttccccctgggcggcgtggccgcccgccccggcttcggcctgagccccatcttccccggcggcgcctgcctgggcaaggcctgcggccgcaagcgcaag

SEQ ID NO: 24 - protein, 786 aa, Homo sapiens
  Elastin (human): UniProtKB - P15502 (ELN_HUMAN); aa 1 - 26 signal peptide; aa 27 - 786 elastin chain
MAGLTAAAPRPGVLLLLLSILHPSRPGGVPGAIPGGVPGGVFYPGAGLGALGGGALGPGGKPLKPVPGGLAGAGLGAGLGAFPAVTFPGALVPGGVADAAAAYKAAKAGAGLGGVPGVGGLGVSAGAVVPQPGAGVKPGKVPGVGLPGVYPGGVLPGARFPGVGVLPGVPTGAGVKPKAPGVGGAFAGIPGVGPFGGPQPGVPLGYPIKAPKLPGGYGLPYTTGKLPYGYGPGGVAGAAGKAGYPTGTGVGPQAAAAAAAKAAAKFGAGAAGVLPGVGGAGVPGVPGAIPGIGGIAGVGTPAAAAAAAAAAKAAKYGAAAGLVPGGPGFGPGVVGVPGAGVPGVGVPGAGIPVVPGAGIPGAAVPGVVSPEAAAKAAAKAAKYGARPGVGVGGIPTYGVGAGGFPGFGVGVGGIPGVAGVPGVGGVPGVGGVPGVGISPEAQAAAAAKAAKYGAAGAGVLGGLVPGAPGAVPGVPGTGGVPGVGTPAAAAAKAAAKAAQFGLVPGVGVAPGVGVAPGVGVAPGVGLAPGVGVAPGVGVAPGVGVAPGIGPGGVAAAAKSAAKVAAKAQLRAAAGLGAGIPGLGVGVGVPGLGVGAGVPGLGVGAGVPGFGAGADEGVRRSLSPELREGDPSSSQHLPSTPSSPRVPGALAAAKAAKYGAAVPGVLGGLGALGGVGIPGGVVGAGPAAAAAAAKAAAKAAQFGLVGAAGLGGLGVGGLGVPGVGGLGGIPPAAAAKAAKYGAAGLGGVLGGAGQFPLGGVAARPGFGLSPIFPGGACLGKACGRKRK

SEQ ID NO: 25 - DNA, 2598 bp, Homo sapiens
  Fibrinogen alpha chain (FGA / human) exemplarily: UniProtKB - P02671 (FIBA_HUMAN), aa 1 - 19 signal peptide; aa 20 - 35 Fibrinopeptide A; 36 - 866 Fibrin Monomer α chain
atgttcagcatgcgcatcgtgtgcctggtgctgagcgtggtgggcaccgcctggaccgccgacagcggcgagggcgacttcctggccgagggcggcggcgtgcgcggcccccgcgtggtggagcgccaccagagcgcctgcaaggacagcgactggcccttctgcagcgacgaggactggaactacaagtgccccagcggctgccgcatgaagggcctgatcgacgaggtgaaccaggacttcaccaaccgcatcaacaagctgaagaacagcctgttcgagtaccagaagaacaacaaggacagccacagcctgaccaccaacatcatggagatcctgcgcggcgacttcagcagcgccaacaaccgcgacaacacctacaaccgcgtgagcgaggacctgcgcagccgcatcgaggtgctgaagcgcaaggtgatcgagaaggtgcagcacatccagctgctgcagaagaacgtgcgcgcccagctggtggacatgaagcgcctggaggtggacatcgacatcaagatccgcagctgccgcggcagctgcagccgcgccctggcccgcgaggtggacctgaaggactacgaggaccagcagaagcagctggagcaggtgatcgccaaggacctgctgcccagccgcgaccgccagcacctgcccctgatcaagatgaagcccgtgcccgacctggtgcccggcaacttcaagagccagctgcagaaggtgccccccgagtggaaggccctgaccgacatgccccagatgcgcatggagctggagcgccccggcggcaacgagatcacccgcggcggcagcaccagctacggcaccggcagcgagaccgagagcccccgcaaccccagcagcgccggcagctggaacagcggcagcagcggccccggcagcaccggcaaccgcaaccccggcagcagcggcaccggcggcaccgccacctggaagcccggcagcagcggccccggcagcaccggcagctggaacagcggcagcagcggcaccggcagcaccggcaaccagaaccccggcagcccccgccccggcagcaccggcacctggaaccccggcagcagcgagcgcggcagcgccggccactggaccagcgagagcagcgtgagcggcagcaccggccagtggcacagcgagagcggcagcttccgccccgacagccccggcagcggcaacgcccgccccaacaaccccgactggggcaccttcgaggaggtgagcggcaacgtgagccccggcacccgccgcgagtaccacaccgagaagctggtgaccagcaagggcgacaaggagctgcgcaccggcaaggagaaggtgaccagcggcagcaccaccaccacccgccgcagctgcagcaagaccgtgaccaagaccgtgatcggccccgacggccacaaggaggtgaccaaggaggtggtgaccagcgaggacggcagcgactgccccgaggccatggacctgggcaccctgagcggcatcggcaccctggacggcttccgccaccgccaccccgacgaggccgccttcttcgacaccgccagcaccggcaagaccttccccggcttcttcagccccatgctgggcgagttcgtgagcgagaccgagagccgcggcagcgagagcggcatcttcaccaacaccaaggagagcagcagccaccaccccggcatcgccgagttccccagccgcggcaagagcagcagctacagcaagcagttcaccagcagcaccagctacaaccgcggcgacagcaccttcgagagcaagagctacaagatggccgacgaggccggcagcgaggccgaccacgagggcacccacagcaccaagcgcggccacgccaagagccgccccgtgcgcgactgcgacgacgtgctgcagacccaccccagcggcacccagagcggcatcttcaacatcaagctgcccggcagcagcaagatcttcagcgtgtactgcgaccaggagaccagcctgggcggctggctgctgatccagcagcgcatggacggcagcctgaacttcaaccgcacctggcaggactacaagcgcggcttcggcagcctgaacgacgagggcgagggcgagttctggctgggcaacgactacctgcacctgctgacccagcgcggcagcgtgctgcgcgtggagctggaggactgggccggcaacgaggcctacgccgagtaccacttccgcgtgggcagcgaggccgagggctacgccctgcaggtgagcagctacgagggcaccgccggcgacgccctgatcgagggcagcgtggaggagggcgccgagtacaccagccacaacaacatgcagttcagcaccttcgaccgcgacgccgaccagtgggaggagaactgcgccgaggtgtacggcggcggctggtggtacaacaactgccaggccgccaacctgaacggcatctactaccccggcggcagctacgacccccgcaacaacagcccctacgagatcgagaacggcgtggtgtgggtgagcttccgcggcgccgactacagcctgcgcgccgtgcgcatgaagatccgccccctggtgacccag

SEQ ID NO: 26 - protein, 866 aa, Homo sapiens
  Fibrinogen alpha chain (FGA / human) exemplarily: UniProtKB - P02671 (FIBA_HUMAN), aa 1 - 19 signal peptide; aa 20 - 35 Fibrinopeptide A; 36 - 866 Fibrin Monomer α chain
MFSMRIVCLVLSVVGTAWTADSGEGDFLAEGGGVRGPRVVERHQSACKDSDWPFCSDEDWNYKCPSGCRMKGLIDEVNQDFTNRINKLKNSLFEYQKNNKDSHSLTTNIMEILRGDFSSANNRDNTYNRVSEDLRSRIEVLKRKVIEKVQHIQLLQKNVRAQLVDMKRLEVDIDIKIRSCRGSCSRALAREVDLKDYEDQQKQLEQVIAKDLLPSRDRQHLPLIKMKPVPDLVPGNFKSQLQKVPPEWKALTDMPQMRMELERPGGNEITRGGSTSYGTGSETESPRNPSSAGSWNSGSSGPGSTGNRNPGSSGTGGTATWKPGSSGPGSTGSWNSGSSGTGSTGNQNPGSPRPGSTGTWNPGSSERGSAGHWTSESSVSGSTGQWHSESGSFRPDSPGSGNARPNNPDWGTFEEVSGNVSPGTRREYHTEKLVTSKGDKELRTGKEKVTSGSTTTTRRSCSKTVTKTVIGPDGHKEVTKEVVTSEDGSDCPEAMDLGTLSGIGTLDGFRHRHPDEAAFFDTASTGKTFPGFFSPMLGEFVSETESRGSESGIFTNTKESSSHHPGIAEFPSRGKSSSYSKQFTSSTSYNRGDSTFESKSYKMADEAGSEADHEGTHSTKRGHAKSRPVRDCDDVLQTHPSGTQSGIFNIKLPGSSKIFSVYCDQETSLGGWLLIQQRMDGSLNFNRTWQDYKRGFGSLNDEGEGEFWLGNDYLHLLTQRGSVLRVELEDWAGNEAYAEYHFRVGSEAEGYALQVSSYEGTAGDALIEGSVEEGAEYTSHNNMQFSTFDRDADQWEENCAEVYGGGWWYNNCQAANLNGIYYPGGSYDPRNNSPYEIENGVVWVSFRGADYSLRAVRMKIRPLVTQ

SEQ ID NO: 27 - DNA, 1755 bp, Homo sapiens
  hsa = recombinant human serum albumin, coding sequence
gacgctcacaaatctgaagttgctcaccgtttcaaagacctgggtgaagaaaacttcaaagctctggttctgatcgctttcgctcagtacctgcagcagtgcccgttcgaagaccacgttaaactggttaacgaagttaccgaatttgctaaaacctgcgttgctgacgaatctgctgaaaactgcgacaaatctctgcacaccctgttcggtgacaaactgtgtaccgttgctaccctgcgtgaaacctacggtgaaatggctgactgctgcgctaaacaggaaccggaacgtaacgaatgcttcctgcagcacaaagacgacaacccgaacctgccgcgtctggttcgtccggaagttgacgttatgtgtaccgctttccacgacaacgaagaaaccttcctgaaaaaatacctgtacgaaatcgctcgtcgtcacccgtacttctacgctccggaactgctgttcttcgctaaacgttacaaagctgctttcaccgaatgctgccaggctgctgacaaagctgcttgcctgctgccgaaactggacgaactgcgtgacgaaggtaaagcgtcttctgctaaacagcgtctgaaatgcgcttctctgcagaaattcggtgaacgtgctttcaaagcgtgggctgttgctcgtctgtctcagcgtttcccgaaagctgaatttgctgaagtttctaaactggttaccgacctgaccaaagttcacaccgaatgctgccacggtgacctgctggaatgcgctgacgaccgtgctgacctggctaaatacatctgcgaaaaccaggactctatctcgtctaaactgaaagaatgctgcgaaaaaccgctgctggaaaaatctcactgcatcgctgaagttgaaaacgacgaaatgccggctgacctgccgtctctggctgctgacttcgttgaatctaaagacgtttgcaaaaactacgctgaagctaaagacgttttcctgggtatgttcctgtacgaatacgctcgtcgtcacccggactactctgttgttctgctgctgcgtctggctaaaacctacgaaaccaccctggaaaaatgctgcgctgctgctgacccgcacgaatgctacgctaaagttttcgacgagttcaaaccgctggttgaagaaccgcagaacctgatcaaacagaactgcgaactgttcgaacagctgggtgaatacaaattccagaacgctctgctggttcgttacaccaaaaaagttccgcaggtttctaccccgaccctggttgaagtttctcgtaacctgggtaaagttggttctaaatgctgcaaacacccggaagctaaacgtatgccgtgcgctgaagactacctgtctgttgttctgaaccagctgtgcgttctgcacgaaaaaaccccggtttctgaccgtgttaccaaatgctgcaccgaatctctggttaaccgtcgtccgtgcttctctgctctggaagttgacgaaacctacgttccgaaagagttcaacgctgaaaccttcaccttccacgctgacatctgcaccctgtctgaaaaagaacgtcagatcaaaaaacagaccgctctggttgaactggttaaacacaaaccgaaagctaccaaagaacagctgaaagctgttatggacgacttcgctgctttcgttgaaaaatgctgcaaagctgacgacaaagaaacctgcttcgctgaagaaggtaaaaaactggttgctgcttctcaggctgctctgggtctg

SEQ ID NO: 28 - protein, 585 aa, Homo sapiens [sequence omitted]

SEQ ID NO: 29 - DNA, 7431 bp, Homo sapiens
atgctgcgcggccccggccccggcctgctgctgctggccgtgcagtgcctgggcaccgccgtgcccagcaccggcgccagcaagagcaagcgccaggcccagcagatggtgcagccccagagccccgtggccgtgagccagagcaagcccggctgctacgacaacggcaagcactaccagatcaaccagcagtgggagcgcacctacctgggcaacgccctggtgtgcacctgctacggcggcagccgcggcttcaactgcgagagcaagcccgaggccgaggagacctgcttcgacaagtacaccggcaacacctaccgcgtgggcgacacctacgagcgccccaaggacagcatgatctgggactgcacctgcatcggcgccggccgcggccgcatcagctgcaccatcgccaaccgctgccacgagggcggccagagctacaagatcggcgacacctggcgccgcccccacgagaccggcggctacatgctggagtgcgtgtgcctgggcaacggcaagggcgagtggacctgcaagcccatcgccgagaagtgcttcgaccacgccgccggcaccagctacgtggtgggcgagacctgggagaagccctaccagggctggatgatggtggactgcacctgcctgggcgagggcagcggccgcatcacctgcaccagccgcaaccgctgcaacgaccaggacacccgcaccagctaccgcatcggcgacacctggagcaagaaggacaaccgcggcaacctgctgcagtgcatctgcaccggcaacggccgcggcgagtggaagtgcgagcgccacaccagcgtgcagaccaccagcagcggcagcggccccttcaccgacgtgcgcgccgccgtgtaccagccccagccccacccccagccccccccctacggccactgcgtgaccgacagcggcgtggtgtacagcgtgggcatgcagtggctgaagacccagggcaacaagcagatgctgtgcacctgcctgggcaacggcgtgagctgccaggagaccgccgtgacccagacctacggcggcaacagcaacggcgagccctgcgtgctgcccttcacctacaacggccgcaccttctacagctgcaccaccgagggccgccaggacggccacctgtggtgcagcaccaccagcaactacgagcaggaccagaagtacagcttctgcaccgaccacaccgtgctggtgcagacccgcggcggcaacagcaacggcgccctgtgccacttccccttcctgtacaacaaccacaactacaccgactgcaccagcgagggccgccgcgacaacatgaagtggtgcggcaccacccagaactacgacgccgaccagaagttcggcttctgccccatggccgcccacgaggagatctgcaccaccaacgagggcgtgatgtaccgcatcggcgaccagtgggacaagcagcacgacatgggccacatgatgcgctgcacctgcgtgggcaacggccgcggcgagtggacctgcatcgcctacagccagctgcgcgaccagtgcatcgtggacgacatcacctacaacgtgaacgacaccttccacaagcgccacgaggagggccacatgctgaactgcacctgcttcggccagggccgcggccgctggaagtgcgaccccgtggaccagtgccaggacagcgagaccggcaccttctaccagatcggcgacagctgggagaagtacgtgcacggcgtgcgctaccagtgctactgctacggccgcggcatcggcgagtggcactgccagcccctgcagacctaccccagcagcagcggccccgtggaggtgttcatcaccgagacccccagccagcccaacagccaccccatccagtggaacgccccccagcccagccacatcagcaagtacatcctgcgctggcgccccaagaacagcgtgggccgctggaaggaggccaccatccccggccacctgaacagctacaccatcaagggcctgaagcccggcgtggtgtacgagggccagctgatcagcatccagcagtacggccaccaggaggtgacccgcttcgacttcaccaccaccagcaccagcacccccgtgaccagcaacaccgtgaccggcgagaccacccccttcagccccctggtggccaccagcgagagcgtgaccgagatcaccgccagcagcttcgtggtgagctgggtgagcgccagcgacaccgtgagcggcttccgcgtggagtacgagctgagcgaggagggcgacgagccccagtacctggacctgcccagcaccgccaccagcgtgaacatccccgacctgctgcccggccgcaagtacatcgtgaacgtgtaccagatcagcgaggacggcgagcagagcctgatcctgagcaccagccagaccaccgcccccgacgccccccccgacaccaccgtggaccaggtggacgacaccagcatcgtggtgcgctggagccgcccccaggcccccatcaccggctaccgcatcgtgtacagccccagcgtggagggcagcagcaccgagctgaacctgcccgagaccgccaacagcgtgaccctgagcgacctgcagcccggcgtgcagtacaacatcaccatctacgccgtggaggagaaccaggagagcacccccgtggtgatccagcaggagaccaccggcaccccccgcagcgacaccgtgcccagcccccgcgacctgcagttcgtggaggtgaccgacgtgaaggtgaccatcatgtggaccccccccgagagcgccgtgaccggctaccgcgtggacgtgatccccgtgaacctgcccggcgagcacggccagcgcctgcccatcagccgcaacaccttcgccgaggtgaccggcctgagccccggcgtgacctactacttcaaggtgttcgccgtgagccacggccgcgagagcaagcccctgaccgcccagcagaccaccaagctggacgcccccaccaacctgcagttcgtgaacgagaccgacagcaccgtgctggtgcgctggacccccccccgcgcccagatcaccggctaccgcctgaccgtgggcctgacccgccgcggccagccccgccagtacaacgtgggccccagcgtgagcaagtaccccctgcgcaacctgcagcccgccagcgagtacaccgtgagcctggtggccatcaagggcaaccaggagagccccaaggccaccggcgtgttcaccaccctgcagcccggcagcagcatccccccctacaacaccgaggtgaccgagaccaccatcgtgatcacctggacccccgccccccgcatcggcttcaagctgggcgtgcgccccagccagggcggcgaggccccccgcgaggtgaccagcgacagcggcagcatcgtggtgagcggcctgacccccggcgtggagtacgtgtacaccatccaggtgctgcgcgacggccaggagcgcgacgcccccatcgtgaacaaggtggtgacccccctgagcccccccaccaacctgcacctggaggccaaccccgacaccggcgtgctgaccgtgagctgggagcgcagcaccacccccgacatcaccggctaccgcatcaccaccacccccaccaacggccagcagggcaacagcctggaggaggtggtgcacgccgaccagagcagctgcaccttcgacaacctgagccccggcctggagtacaacgtgagcgtgtacaccgtgaaggacgacaaggagagcgtgcccatcagcgacaccatcatccccgaggtgccccagctgaccgacctgagcttcgtggacatcaccgacagcagcatcggcctgcgctggacccccctgaacagcagcaccatcatcggctaccgcatcaccgtggtggccgccggcgagggcatccccatcttcgaggacttcgtggacagcagcgtgggctactacaccgtgaccggcctggagcccggcatcgactacgacatcagcgtgatcaccctgatcaacggcggcgagagcgcccccaccaccctgacccagcagaccgccgtgcccccccccaccgacctgcgcttcaccaacatcggccccgacaccatgcgcgtgacctgggcccccccccccagcatcgacctgaccaacttcctggtgcgctacagccccgtgaagaacgaggaggacgtggccgagctgagcatcagccccagcgacaacgccgtggtgctgaccaacctgctgcccggcaccgagtacgtggtgagcgtgagcagcgtgtacgagcagcacgagagcacccccctgcgcggccgccagaagaccggcctggacagccccaccggcatcgacttcagcgacatcaccgccaacagcttcaccgtgcactggatcgccccccgcgccaccatcaccggctaccgcatccgccaccaccccgagcacttcagcggccgcccccgcgaggaccgcgtgccccacagccgcaacagcatcaccctgaccaacctgacccccggcaccgagtacgtggtgagcatcgtggccctgaacggccgcgaggagagccccctgctgatcggccagcagagcaccgtgagcgacgtgccccgcgacctggaggtggtggccgccacccccaccagcctgctgatcagctgggacgcccccgccgtgaccgtgcgctactaccgcatcacctacggcgagaccggcggcaacagccccgtgcaggagttcaccgtgcccggcagcaagagcaccgccaccatcagcggcctgaagcccggcgtggactacaccatcaccgtgtacgccgtgaccggccgcggcgacagccccgccagcagcaagcccatcagcatcaactaccgcaccgagatcgacaagcccagccagatgcaggtgaccgacgtgcaggacaacagcatcagcgtgaagtggctgcccagcagcagccccgtgaccggctaccgcgtgaccaccacccccaagaacggccccggccccaccaagaccaagaccgccggccccgaccagaccgagatgaccatcgagggcctgcagcccaccgtggagtacgtggtgagcgtgtacgcccagaaccccagcggcgagagccagcccctggtgcagaccgccgtgaccaacatcgaccgccccaagggcctggccttcaccgacgtggacgtggacagcatcaagatcgcctgggagagcccccagggccaggtgagccgctaccgcgtgacctacagcagccccgaggacggcatccacgagctgttccccgcccccgacggcgaggaggacaccgccgagctgcagggcctgcgccccggcagcgagtacaccgtgagcgtggtggccctgcacgacgacatggagagccagcccctgatcggcacccagagcaccgccatccccgcccccaccgacctgaagttcacccaggtgacccccaccagcctgagcgcccagtggaccccccccaacgtgcagctgaccggctaccgcgtgcgcgtgacccccaaggagaagaccggccccatgaaggagatcaacctggcccccgacagcagcagcgtggtggtgagcggcctgatggtggccaccaagtacgaggtgagcgtgtacgccctgaaggacaccctgaccagccgccccgcccagggcgtggtgaccaccctggagaacgtgagccccccccgccgcgcccgcgtgaccgacgccaccgagaccaccatcaccatcagctggcgcaccaagaccgagaccatcaccggcttccaggtggacgccgtgcccgccaacggccagacccccatccagcgcaccatcaagcccgacgtgcgcagctacaccatcaccggcctgcagcccggcaccgactacaagatctacctgtacaccctgaacgacaacgcccgcagcagccccgtggtgatcgacgccagcaccgccatcgacgcccccagcaacctgcgcttcctggccaccacccccaacagcctgctggtgagctggcagcccccccgcgcccgcatcaccggctacatcatcaagtacgagaagcccggcagccccccccgcgaggtggtgccccgcccccgccccggcgtgaccgaggccaccatcaccggcctggagcccggcaccgagtacaccatctacgtgatcgccctgaagaacaaccagaagagcgagcccctgatcggccgcaagaagaccgacgagctgccccagctggtgaccctgccccaccccaacctgcacggccccgagatcctggacgtgcccagcaccgtgcagaagacccccttcgtgacccaccccggctacgacaccggcaacggcatccagctgcccggcaccagcggccagcagcccagcgtgggccagcagatgatcttcgaggagcacggcttccgccgcaccaccccccccaccaccgccacccccatccgccaccgcccccgcccctacccccccaacgtgggcgaggagatccagatcggccacatcccccgcgaggacgtggactaccacctgtacccccacggccccggcctgaaccccaacgccagcaccggccaggaggccctgagccagaccaccatcagctgggcccccttccaggacaccagcgagtacatcatcagctgccaccccgtgggcaccgacgaggagcccctgcagttccgcgtgcccggcaccagcaccagcgccaccctgaccggcctgacccgcggcgccacctacaacgtgatcgtggaggccctgaaggaccagcagcgccacaaggtgcgcgaggaggtggtgaccgtgggcaacagcgtgaacgagggcctgaaccagcccaccgacgacagctgcttcgacccctacaccgtgagccactacgccgtgggcgacgagtgggagcgcatgagcgagagcggcttcaagctgctgtgccagtgcctgggcttcggcagcggccacttccgctgcgacagcagccgctggtgccacgacaacggcgtgaactacaagatcggcgagaagtgggaccgccagggcgagaacggccagatgatgagctgcacctgcctgggcaacggcaagggcgagttcaagtgcgacccccacgaggccacctgctacgacgacggcaagacctaccacgtgggcgagcagtggcagaaggagtacctgggcgccatctgcagctgcacctgcttcggcggccagcgcggctggcgctgcgacaactgccgccgccccggcggcgagcccagccccgagggcaccaccggccagagctacaaccagtacagccagcgctaccaccagcgcaccaacaccaacgtgaactgccccatcgagtgcttcatgcccctggacgtgcaggccgaccgcgaggacagccgcgag

SEQ ID NO: 30 - protein, 2477 aa, Homo sapiens
  Fibronectin / FN1 (human): UniProtKB - P02751 (FINC_HUMAN), aa 1 - 31 signal peptide; aa 32 - 2477 fibronectin chain combined DNA/RNA molecule
MLRGPGPGLLLLAVQCLGTAVPSTGASKSKRQAQQMVQPQSPVAVSQSKPGCYDNGKHYQINQQWERTYLGNALVCTCYGGSRGFNCESKPEAEETCFDKYTGNTYRVGDTYERPKDSMIWDCTCIGAGRGRISCTIANRCHEGGQSYKIGDTWRRPHETGGYMLECVCLGNGKGEWTCKPIAEKCFDHAAGTSYVVGETWEKPYQGWMMVDCTCLGEGSGRITCTSRNRCNDQDTRTSYRIGDTWSKKDNRGNLLQCICTGNGRGEWKCERHTSVQTTSSGSGPFTDVRAAVYQPQPHPQPPPYGHCVTDSGVVYSVGMQWLKTQGNKQMLCTCLGNGVSCQETAVTQTYGGNSNGEPCVLPFTYNGRTFYSCTTEGRQDGHLWCSTTSNYEQDQKYSFCTDHTVLVQTRGGNSNGALCHFPFLYNNHNYTDCTSEGRRDNMKWCGTTQNYDADQKFGFCPMAAHEEICTTNEGVMYRIGDQWDKQHDMGHMMRCTCVGNGRGEWTCIAYSQLRDQCIVDDITYNVNDTFHKRHEEGHMLNCTCFGQGRGRWKCDPVDQCQDSETGTFYQIGDSWEKYVHGVRYQCYCYGRGIGEWHCQPLQTYPSSSGPVEVFITETPSQPNSHPIQWNAPQPSHISKYILRWRPKNSVGRWKEATIPGHLNSYTIKGLKPGVVYEGQLISIQQYGHQEVTRFDFTTTSTSTPVTSNTVTGETTPFSPLVATSESVTEITASSFVVSWVSASDTVSGFRVEYELSEEGDEPQYLDLPSTATSVNIPDLLPGRKYIVNVYQISEDGEQSLILSTSQTTAPDAPPDTTVDQVDDTSIVVRWSRPQAPITGYRIVYSPSVEGSSTELNLPETANSVTLSDLQPGVQYNITIYAVEENQESTPVVIQQETTGTPRSDTVPSPRDLQFVEVTDVKVTIMWTPPESAVTGYRVDVIPVNLPGEHGQRLPISRNTFAEVTGLSPGVTYYFKVFAVSHGRESKPLTAQQTTKLDAPTNLQFVNETDSTVLVRWTPPRAQITGYRLTVGLTRRGQPRQYNVGPSVSKYPLRNLQPASEYTVSLVAIKGNQESPKATGVFTTLQPGSSIPPYNTEVTETTIVITWTPAPRIGFKLGVRPSQGGEAPREVTSDSGSIVVSGLTPGVEYVYTIQVLRDGQERDAPIVNKVVTPLSPPTNLHLEANPDTGVLTVSWERSTTPDITGYRITTTPTNGQQGNSLEEVVHADQSSCTFDNLSPGLEYNVSVYTVKDDKESVPISDTIIPEVPQLTDLSFVDITDSSIGLRWTPLNSSTIIGYRITVVAAGEGIPIFEDFVDSSVGYYTVTGLEPGIDYDISVITLINGGESAPTTLTQQTAVPPPTDLRFTNIGPDTMRVTWAPPPSIDLTNFLVRYSPVKNEEDVAELSISPSDNAVVLTNLLPGTEYVVSVSSVYEQHESTPLRGRQKTGLDSPTGIDFSDITANSFTVHWIAPRATITGYRIRHHPEHFSGRPREDRVPHSRNSITLTNLTPGTEYVVSIVALNGREESPLLIGQQSTVSDVPRDLEVVAATPTSLLISWDAPAVTVRYYRITYGETGGNSPVQEFTVPGSKSTATISGLKPGVDYTITVYAVTGRGDSPASSKPISINYRTEIDKPSQMQVTDVQDNSISVKWLPSSSPVTGYRVTTTPKNGPGPTKTKTAGPDQTEMTIEGLQPTVEYVVSVYAQNPSGESQPLVQTAVTNIDRPKGLAFTDVDVDSIKIAWESPQGQVSRYRVTYSSPEDGIHELFPAPDGEEDTAELQGLRPGSEYTVSVVALHDDMESQPLIGTQSTAIPAPTDLKFTQVTPTSLSAQWTPPNVQLTGYRVRVTPKEKTGPMKEINLAPDSSSVVVSGLMVATKYEVSVYALKDTLTSRPAQGVVTTLENVSPPRRARVTDATETTITISWRTKTETITGFQVDAVPANGQTPIQRTIKPDVRSYTITGLQPGTDYKIYLYTLNDNARSSPVVIDASTAIDAPSNLRFLATTPNSLLVSWQPPRARITGYIIKYEKPGSPPREVVPRPRPGVTEATITGLEPGTEYTIYVIALKNNQKSEPLIGRKKTDELPQLVTLPHPNLHGPEILDVPSTVQKTPFVTHPGYDTGNGIQLPGTSGQQPSVGQQMIFEEHGFRRTTPPTTATPIRHRPRPYPPNVGEEIQIGHIPREDVDYHLYPHGPGLNPNASTGQEALSQTTISWAPFQDTSEYIISCHPVGTDEEPLQFRVPGTSTSATLTGLTRGATYNVIVEALKDQQRHKVREEVVTVGNSVNEGLNQPTDDSCFDPYTVSHYAVGDEWERMSESGFKLLCQCLGFGSGHFRCDSSRWCHDNGVNYKIGEKWDRQGENGQMMSCTCLGNGKGEFKCDPHEATCYDDGKTYHVGEQWQKEYLGAICSCTCFGGQRGWRCDNCRRPGGEPSPEGTTGQSYNQYSQRYHQRTNTNVNCPIECFMPLDVQADREDSRE

SEQ ID NO: 31 - DNA, 450 bp, Artificial Sequence
  recombinant resilin (10x), coding sequence
ggtggtcgaccttctgattcttacggtgctcctggtggtggtaatggtggtcgaccttctgattcttacggtgctcctggtggtggtaatggtggtcgaccttctgattcttacggtgctcctggtggtggtaatggtggtcgaccttctgattcttacggtgctcctggtggtggtaatggtggtcgaccttctgattcttacggtgctcctggtggtggtaatggtggtcgaccttctgattcttacggtgctcctggtggtggtaatggtggtcgaccttctgattcttacggtgctcctggtggtggtaatggtggtcgaccttctgattcttacggtgctcctggtggtggtaatggtggtcgaccttctgattcttacggtgctcctggtggtggtaatggtggtcgaccttctgattcttacggtgctcctggtggtggtaat

SEQ ID NO: 32 - protein, 150 aa, Artificial Sequence
  recombinant resilin (10x),
GGRPSDSYGAPGGGNGGRPSDSYGAPGGGNGGRPSDSYGAPGGGNGGRPSDSYGAPGGGNGGRPSDSYGAPGGGNGGRPSDSYGAPGGGNGGRPSDSYGAPGGGNGGRPSDSYGAPGGGNGGRPSDSYGAPGGGNGGRPSDSYGAPGGGN

SEQ ID NO: 33 - DNA, 1050 bp, Artificial Sequence
  spisi10 = recombinant spider silk 10x
ggtcgtggtggtctgggtggtcagggtgctggtatggctgctgctgctgctatgggtggtgctggtcagggtggttacggtggtctgggttctcagggtacctctggtcgtggtggtctgggtggtcagggtgctggtatggctgctgctgctgctatgggtggtgctggtcagggtggttacggtggtctgggttctcagggtacctctggtcgtggtggtctgggtggtcagggtgctggtatggctgctgctgctgctatgggtggtgctggtcagggtggttacggtggtctgggttctcagggtacctctggtcgtggtggtctgggtggtcagggtgctggtatggctgctgctgctgctatgggtggtgctggtcagggtggttacggtggtctgggttctcagggtacctctggtcgtggtggtctgggtggtcagggtgctggtatggctgctgctgctgctatgggtggtgctggtcagggtggttacggtggtctgggttctcagggtacctctggtcgtggtggtctgggtggtcagggtgctggtatggctgctgctgctgctatgggtggtgctggtcagggtggttacggtggtctgggttctcagggtacctctggtcgtggtggtctgggtggtcagggtgctggtatggctgctgctgctgctatgggtggtgctggtcagggtggttacggtggtctgggttctcagggtacctctggtcgtggtggtctgggtggtcagggtgctggtatggctgctgctgctgctatgggtggtgctggtcagggtggttacggtggtctgggttctcagggtacctctggtcgtggtggtctgggtggtcagggtgctggtatggctgctgctgctgctatgggtggtgctggtcagggtggttacggtggtctgggttctcagggtacctctggtcgtggtggtctgggtggtcagggtgctggtatggctgctgctgctgctatgggtggtgctggtcagggtggttacggtggtctgggttctcagggtacctct

SEQ ID NO: 34 - protein, 350 aa, Artificial Sequence
  spisi10 = recombinant spider silk 10x
GRGGLGGQGAGMAAAAAMGGAGQGGYGGLGSQGTSGRGGLGGQGAGMAAAAAMGGAGQGGYGGLGSQGTSGRGGLGGQGAGMAAAAAMGGAGQGGYGGLGSQGTSGRGGLGGQGAGMAAAAAMGGAGQGGYGGLGSQGTSGRGGLGGQGAGMAAAAAMGGAGQGGYGGLGSQGTSGRGGLGGQGAGMAAAAAMGGAGQGGYGGLGSQGTSGRGGLGGQGAGMAAAAAMGGAGQGGYGGLGSQGTSGRGGLGGQGAGMAAAAAMGGAGQGGYGGLGSQGTSGRGGLGGQGAGMAAAAAMGGAGQGGYGGLGSQGTSGRGGLGGQGAGMAAAAAMGGAGQGGYGGLGSQGTS

SEQ ID NO: 35 - DNA, 720 bp, Unknown
  mEGFP
ggtatggtgagcaagggcgaggagctgttcaccggggtggtgcccatcctggtcgagctggacggcgacgtaaacggccacaagttcagcgtgtccggcgagggcgagggcgatgccacctacggcaagctgaccctgaagttcatctgcaccaccggcaagctgcccgtgccctggcccaccctcgtgaccaccctgacctacggcgtgcagtgcttcagccgctaccccgaccacatgaagcagcacgacttcttcaagtccgccatgcccgaaggctacgtccaggagcgcaccatcttcttcaaggacgacggcaactacaagacccgcgccgaggtgaagttcgagggcgacaccctggtgaaccgcatcgagctgaagggcatcgacttcaaggaggacggcaacatcctggggcacaagctggagtacaactacaacagccacaacgtctatatcatggccgacaagcagaagaacggcatcaaggtgaacttcaagatccgccacaacatcgaggacggcagcgtgcagctcgccgaccactaccagcagaacacccccatcggcgacggccccgtgctgctgcccgacaaccactacctgagcacccagtccaagctgagcaaagaccccaacgagaagcgcgatcacatggtcctgctggagttcgtgaccgccgccgggatcactctcggcatggacgagctgtacaag

SEQ ID NO: 36 - protein, 239 aa, Unknown
  mEGFP
GMVSKGEELFTGVVPILVELDGDVNGHKFSVSGEGEGDATYGKLTLKFICTTGKLPVPWPTLVTTLTYGVQCFSRYPDHMKQHDFFKSAMPEGYVQERTIFFKDDGNYKTRAEVKFEGDTLVNRIELKGIDFKEDGNILGHKLEYNYNSHNVYIMADKQKNGIKVNFKIRHNIEDGSVQLADHYQQNTPIGDGPVLLPDNHYLSTQSKLSKDPNEKRDHMVLLEFVTAAGITLGMDELY

SEQ ID NO: 37 - DNA, 255 bp, Unknown
  SpyCatcher protein
tcaggtgatagtgctacccatattaaattctcaaaacgtgatgaggacggcaaagagttagctggtgcaactatggagttgcgtgattcatctggtaaaactattagtacatggatttcagatggacaagtgaaagatttctacctgtatccaggaaaatatacatttgtcgaaaccgcagcaccagacggttatgaggtagcaactgctattacctttacagttaatgagcaaggtcaggttactgtaaatggc

SEQ ID NO: 38 - protein, 85 aa, Unknown
  SpyCatcher protein
SGDSATHIKFSKRDEDGKELAGATMELRDSSGKTISTWISDGQVKDFYLYPGKYTFVETAAPDGYEVATAITFTVNEQGQVTVNG

SEQ ID NO: 39 - DNA, 714 bp, Aequorea victoria
  Green Fluorescent Protein (Aequorea victoria / Jellyfish): UniProtKB - P42212 (GFP_AEQVI), Green Fluorescent Protein (Aequorea victoria / Jellyfish): UniProtKB - P42212 (GFP_AEQVI), aa 1 - 238 Green fluorescent protein
atgtctaaaggtgaagaactgttcaccggtgttgttccgatcctggttgaactggacggtgacgttaacggtcacaaattctctgtttctggtgaaggtgaaggtgacgctacctacggtaaactgaccctgaaattcatctgcaccaccggtaaactgccggttccgtggccgaccctggttaccaccttctcttacggtgttcagtgcttctctcgttacccggaccacatgaaacagcacgacttcttcaaatctgctatgccggaaggttacgttcaggaacgtaccatcttcttcaaagacgacggtaactacaaaacccgtgctgaagttaaattcgaaggtgacaccctggttaaccgtatcgaactgaaaggtatcgacttcaaagaagacggtaacatcctgggtcacaaactggaatacaactacaactctcacaacgtttacatcatggctgacaaacagaaaaacggtatcaaagttaacttcaaaatccgtcacaacatcgaagacggttctgttcagctggctgaccactaccagcagaacaccccgatcggtgacggtccggttctgctgccggacaaccactacctgtctacccagtctgctctgtctaaagacccgaacgaaaaacgtgaccacatggttctgctggaattcgttaccgctgctggtatcacccacggtatggacgaactgtacaaa

SEQ ID NO: 40 - protein, 238 aa, Aequorea victoria
  Green Fluorescent Protein (Aequorea victoria / Jellyfish): UniProtKB - P42212 (GFP_AEQVI), Green Fluorescent Protein (Aequorea victoria / Jellyfish): UniProtKB - P42212 (GFP_AEQVI), aa 1 - 238 Green fluorescent protein
MSKGEELFTGVVPILVELDGDVNGHKFSVSGEGEGDATYGKLTLKFICTTGKLPVPWPTLVTTFSYGVQCFSRYPDHMKQHDFFKSAMPEGYVQERTIFFKDDGNYKTRAEVKFEGDTLVNRIELKGIDFKEDGNILGHKLEYNYNSHNVYIMADKQKNGIKVNFKIRHNIEDGSVQLADHYQQNTPIGDGPVLLPDNHYLSTQSALSKDPNEKRDHMVLLEFVTAAGITHGMDELYK

SEQ ID NO: 41 - DNA, 1452 bp, Artificial Sequence
  mCHR-TEVrec-mEGFP; mCHR = monomeric mCherry; TEVrec = TEV protease recognition sequence
ggtatggtgagcaagggcgaggaggataacatggccatcatcaaggagttcatgcgcttcaaggtgcacatggagggctccgtgaacggccacgagttcgagatcgagggcgagggcgagggccgcccctacgagggcacccagaccgccaagctgaaggtgaccaagggtggccccctgcccttcgcctgggacatcctgtcccctcagttcatgtacggctccaaggcctacgtgaagcaccccgccgacatccccgactacttgaagctgtccttccccgagggcttcaagtgggagcgcgtgatgaacttcgaggacggcggcgtggtgaccgtgacccaggactcctccctgcaggacggcgagttcatctacaaggtgaagctgcgcggcaccaacttcccctccgacggccccgtaatgcagaagaagaccatgggctgggaggcctcctccgagcggatgtaccccgaggacggcgccctgaagggcgagatcaagcagaggctgaagctgaaggacggcggccactacgacgctgaggtcaagaccacctacaaggccaagaagcccgtgcagctgcccggcgcctacaacgtcaacatcaagttggacatcacctcccacaacgaggactacaccatcgtggaacagtacgaacgcgccgagggccgccactccaccggcggcatggacgagctgtacaagggtgaaaacctgtactttcagggtatggtgagcaagggcgaggagctgttcaccggggtggtgcccatcctggtcgagctggacggcgacgtaaacggccacaagttcagcgtgtccggcgagggcgagggcgatgccacctacggcaagctgaccctgaagttcatctgcaccaccggcaagctgcccgtgccctggcccaccctcgtgaccaccctgacctacggcgtgcagtgcttcagccgctaccccgaccacatgaagcagcacgacttcttcaagtccgccatgcccgaaggctacgtccaggagcgcaccatcttcttcaaggacgacggcaactacaagacccgcgccgaggtgaagttcgagggcgacaccctggtgaaccgcatcgagctgaagggcatcgacttcaaggaggacggcaacatcctggggcacaagctggagtacaactacaacagccacaacgtctatatcatggccgacaagcagaagaacggcatcaaggtgaacttcaagatccgccacaacatcgaggacggcagcgtgcagctcgccgaccactaccagcagaacacccccatcggcgacggccccgtgctgctgcccgacaaccactacctgagcacccagtccaagctgagcaaagaccccaacgagaagcgcgatcacatggtcctgctggagttcgtgaccgccgccgggatcactctcggcatggacgagctgtacaag

SEQ ID NO: 42 - protein, 484 aa, Artificial Sequence
  mCHR-TEVrec-mEGFP; mCHR = monomeric mCherry; TEVrec = TEV protease recognition sequence
GMVSKGEEDNMAIIKEFMRFKVHMEGSVNGHEFEIEGEGEGRPYEGTQTAKLKVTKGGPLPFAWDILSPQFMYGSKAYVKHPADIPDYLKLSFPEGFKWERVMNFEDGGVVTVTQDSSLQDGEFIYKVKLRGTNFPSDGPVMQKKTMGWEASSERMYPEDGALKGEIKQRLKLKDGGHYDAEVKTTYKAKKPVQLPGAYNVNIKLDITSHNEDYTIVEQYERAEGRHSTGGMDELYKGENLYFQGMVSKGEELFTGVVPILVELDGDVNGHKFSVSGEGEGDATYGKLTLKFICTTGKLPVPWPTLVTTLTYGVQCFSRYPDHMKQHDFFKSAMPEGYVQERTIFFKDDGNYKTRAEVKFEGDTLVNRIELKGIDFKEDGNILGHKLEYNYNSHNVYIMADKQKNGIKVNFKIRHNIEDGSVQLADHYQQNTPIGDGPVLLPDNHYLSTQSKLSKDPNEKRDHMVLLEFVTAAGITLGMDELYK

SEQ ID NO: 43 - protein, 5 aa, Artificial Sequence
  generic ELP as linker sequence
  VARIANT 4: /NOTE="Xaa = any amino acid
VPGXG

SEQ ID NO: 44 - protein, 5 aa, Artificial Sequence
  Elastin like peptide (ELP) variant
VPGEG

SEQ ID NO: 45 - protein, 5 aa, Artificial Sequence
  Elastin like peptide (ELP) variant
VPGDG

SEQ ID NO: 46 - protein, 5 aa, Artificial Sequence
  Elastin like peptide (ELP) variant
VPGRG

SEQ ID NO: 47 - protein, 5 aa, Artificial Sequence
  Elastin like peptide (ELP) variant
VPGVG

SEQ ID NO: 48 - protein, 5 aa, Artificial Sequence
  Elastin like peptide (ELP) variant
VPGKG

SEQ ID NO: 49 - protein, 5 aa, Artificial Sequence
  Elastin like peptide (ELP) variant
VPGHG

SEQ ID NO: 50 - protein, 5 aa, Artificial Sequence
  Elastin like peptide (ELP) variant
VPGSG

SEQ ID NO: 51 - protein, 5 aa, Artificial Sequence
  Elastin like peptide (ELP) variant
VPGTG

SEQ ID NO: 52 - protein, 5 aa, Artificial Sequence
  Elastin like peptide (ELP) variant
VPGNG

SEQ ID NO: 53 - protein, 5 aa, Artificial Sequence
  Elastin like peptide (ELP) variant
VPGQG

SEQ ID NO: 54 - protein, 5 aa, Artificial Sequence
  Elastin like peptide (ELP) variant
VPGYG

SEQ ID NO: 55 - protein, 5 aa, Artificial Sequence
  Elastin like peptide (ELP) variant
VPGCG

SEQ ID NO: 56 - protein, 5 aa, Artificial Sequence
  Elastin like peptide (ELP) variant
VPGFG

SEQ ID NO: 57 - protein, 5 aa, Artificial Sequence
  Elastin like peptide (ELP) variant
VPGIG

SEQ ID NO: 58 - protein, 5 aa, Artificial Sequence
  Elastin like peptide (ELP) variant
VPGLG

SEQ ID NO: 59 - protein, 5 aa, Artificial Sequence
  Elastin like peptide (ELP) variant
VPGMG

SEQ ID NO: 60 - protein, 5 aa, Artificial Sequence
  Elastin like peptide (ELP) variant
VPGWG

SEQ ID NO: 61 - protein, 5 aa, Artificial Sequence
  Elastin like peptide (ELP) variant
VPGAG

SEQ ID NO: 62 - protein, 5 aa, Artificial Sequence
  Elastin like peptide (ELP) variant
VPGGG

SEQ ID NO: 63 - protein, 15 aa, Artificial Sequence
  Elastin like peptide (ELP) ("DSY")
VPGDGVPGSGVPGYG

SEQ ID NO: 64 - protein, 15 aa, Artificial Sequence
  Elastin like peptide (ELP) ("VRY")
VPGVGVPGRGVPGYG

SEQ ID NO: 65 - protein, 15 aa, Artificial Sequence
  Elastin like peptide (ELP) ("V2Y")
VPGVPVPGVPVPGYG

SEQ ID NO: 66 - protein, 6 aa, Artificial Sequence
  fusion peptide linker (FPL)
DPMSSS

SEQ ID NO: 67 - protein, 7 aa, Artificial Sequence
  fusion peptide linker (FPL)
GGREASS

SEQ ID NO: 68 - protein, 5 aa, Artificial Sequence
  REPEAT 1: /NOTE="number of repetitions = 1-4"
  REPEAT 1..5: repeat of entire sequence
  fusion peptide linker (FPL)
GGGGS

SEQ ID NO: 69 - protein, 5 aa, Artificial Sequence
  fusion peptide linker (FPL)
GGGGG

SEQ ID NO: 70 - protein, 6 aa, Artificial Sequence
  fusion peptide linker (FPL)
GGGGGG

SEQ ID NO: 71 - protein, 8 aa, Artificial Sequence
  fusion peptide linker (FPL)
GGGGGGGG

SEQ ID NO: 72 - protein, 5 aa, Artificial Sequence
  REPEAT 1..5: /NOTE="number of repetitions = 1-4"
  fusion peptide linker (FPL)
EAAAK

SEQ ID NO: 73 - protein, 46 aa, Artificial Sequence
  fusion peptide linker (FPL)
AEAAAKEAAAKEAAAKEAAAKALEAEAAAKEAAAKEAAAKEAAAKA

SEQ ID NO: 74 - protein, 5 aa, Artificial Sequence
  fusion peptide linker (FPL)
PAPAP

SEQ ID NO: 75 - protein, 12 aa, Artificial Sequence
  fusion peptide linker (FPL)
AEAAAKEAAAKA

SEQ ID NO: 76 - protein, 17 aa, Artificial Sequence
  fusion peptide linker (FPL)
VSQTSKLTRAETVFPDV

SEQ ID NO: 77 - protein, 6 aa, Artificial Sequence
  fusion peptide linker (FPL)
PLGLWA

SEQ ID NO: 78 - protein, 6 aa, Artificial Sequence
  fusion peptide linker (FPL)
RVLAEA

SEQ ID NO: 79 - protein, 10 aa, Artificial Sequence
  fusion peptide linker (FPL)
EDVVCCSMSY

SEQ ID NO: 80 - protein, 8 aa, Artificial Sequence
  fusion peptide linker (FPL)
GGIEGRGS

SEQ ID NO: 81 - protein, 10 aa, Artificial Sequence
  fusion peptide linker (FPL)
TRHRQPRGWE

SEQ ID NO: 82 - protein, 10 aa, Artificial Sequence
  fusion peptide linker (FPL)
AGNRVRRSVG

SEQ ID NO: 83 - protein, 9 aa, Artificial Sequence
  fusion peptide linker (FPL)
RRRRRRRRR

SEQ ID NO: 84 - protein, 6 aa, Artificial Sequence
  fusion peptide linker (FPL)
GFLGLE

SEQ ID NO: 85 - protein, 7 aa, Artificial Sequence
  fusion peptide linker (FPL) and protease recognition/cleavage site
  VARIANT 7: /NOTE="Xaa = G or S
ENLYFQX

SEQ ID NO: 86 - protein, 274 aa, Artificial Sequence
  Fusionprotein ULD-(VPGVG)10-ULD
MDPMSSSGTMLPVFCVVEHYENAIEYDCKEEHAEFVLVRKDMLFNQLIEMALLSLGYSHSSAAQAKGLIQVGKWNPVPLSYVTDAPDATVADMLQDVYHVVTLKIQLHSGVPGVGVPGVGVPGVGVPGVGVPGVGVPGVGVPGVGVPGVGVPGVGVPGVGTMLPVFCVVEHYENAIEYDCKEEHAEFVLVRKDMLFNQLIEMALLSLGYSHSSAAQAKGLIQVGKWNPVPLSYVTDAPDATVADMLQDVYHVVTLKIQLHSGGREASSHHHHHH

SEQ ID NO: 87 - DNA, 975 bp, Artificial Sequence
  Fusionprotein ULD-(VPGVG)20-ULD coding sequence
atggatcctatgagctcttctggtaccatgctgccggttttctgcgttgttgaacactacgaaaacgctatcgaatacgactgcaaagaagaacacgctgaatttgttctggttcgtaaagacatgctgttcaaccagctgatcgaaatggctctgctgtctctgggttactctcacagctctgctgctcaggctaaaggtctgatccaggttggtaaatggaacccggttccgctgtcttacgttaccgacgctccggacgctaccgttgctgacatgctgcaggacgtttaccacgttgttaccctgaaaatccagctgcactctggtgttccgggtagaggtgttccgggtagaggtgttccgggtagaggtgttccgggtagaggtgttccgggtagaggtgttccgggtagaggtgttccgggtagaggtgttccgggtagaggtgttccgggtagaggtgttccgggtagaggtgttccgggtagaggtgttccgggtagaggtgttccgggtagaggtgttccgggtagaggtgttccgggtagaggtgttccgggtagaggtgttccgggtagaggtgttccgggtagaggtgttccgggtagaggtgttccgggtagaggtaccatgctgccggttttctgcgttgttgaacactacgaaaacgctatcgaatacgactgcaaagaagaacacgctgaatttgttctggttcgtaaagacatgctgttcaaccagctgatcgaaatggctctgctgtctctgggttactctcacagctctgctgctcaggctaaaggtctgatccaggttggtaaatggaacccggttccgctgtcttacgttaccgacgctccggacgctaccgttgctgacatgctgcaggacgtttaccacgttgttaccctgaaaatccagctgcactctggtggaagagaagcttcatcacaccaccaccaccaccactga

SEQ ID NO: 88 - protein, 324 aa, Artificial Sequence
  Fusionprotein ULD-(VPGVG)20-ULD
MDPMSSSGTMLPVFCVVEHYENAIEYDCKEEHAEFVLVRKDMLFNQLIEMALLSLGYSHSSAAQAKGLIQVGKWNPVPLSYVTDAPDATVADMLQDVYHVVTLKIQLHSGVPGRGVPGRGVPGRGVPGRGVPGRGVPGRGVPGRGVPGRGVPGRGVPGRGVPGRGVPGRGVPGRGVPGRGVPGRGVPGRGVPGRGVPGRGVPGRGVPGRGTMLPVFCVVEHYENAIEYDCKEEHAEFVLVRKDMLFNQLIEMALLSLGYSHSSAAQAKGLIQVGKWNPVPLSYVTDAPDATVADMLQDVYHVVTLKIQLHSGGREASSHHHHHH

SEQ ID NO: 89 - DNA, 1275 bp, Artificial Sequence
  Fusionprotein ULD-(VPGVG)40-ULD coding sequence
atggatcctatgagctcttctggtaccatgctgccggttttctgcgttgttgaacactacgaaaacgctatcgaatacgactgcaaagaagaacacgctgaatttgttctggttcgtaaagacatgctgttcaaccagctgatcgaaatggctctgctgtctctgggttactctcacagctctgctgctcaggctaaaggtctgatccaggttggtaaatggaacccggttccgctgtcttacgttaccgacgctccggacgctaccgttgctgacatgctgcaggacgtttaccacgttgttaccctgaaaatccagctgcactctggtgttccgggtgttggtgttccgggtgttggtgttccgggtgttggtgttccgggtgttggtgttccgggtgttggtgttccgggtgttggtgttccgggtgttggtgttccgggtgttggtgttccgggtgttggtgttccgggtgttggtgttccgggtgttggtgttccgggtgttggtgttccgggtgttggtgttccgggtgttggtgttccgggtgttggtgttccgggtgttggtgttccgggtgttggtgttccgggtgttggtgttccgggtgttggtgttccgggtgttggtgttccgggtgttggtgttccgggtgttggtgttccgggtgttggtgttccgggtgttggtgttccgggtgttggtgttccgggtgttggtgttccgggtgttggtgttccgggtgttggtgttccgggtgttggtgttccgggtgttggtgttccgggtgttggtgttccgggtgttggtgttccgggtgttggtgttccgggtgttggtgttccgggtgttggtgttccgggtgttggtgttccgggtgttggtgttccgggtgttggtgttccgggtgttggtgttccgggtgttggtaccatgctgccggttttctgcgttgttgaacactacgaaaacgctatcgaatacgactgcaaagaagaacacgctgaatttgttctggttcgtaaagacatgctgttcaaccagctgatcgaaatggctctgctgtctctgggttactctcacagctctgctgctcaggctaaaggtctgatccaggttggtaaatggaacccggttccgctgtcttacgttaccgacgctccggacgctaccgttgctgacatgctgcaggacgtttaccacgttgttaccctgaaaatccagctgcactctggtggaagagaagcttcatcacaccaccaccaccaccactga

SEQ ID NO: 90 - protein, 424 aa, Artificial Sequence
  Fusionprotein ULD-(VPGVG)40-ULD
MDPMSSSGTMLPVFCVVEHYENAIEYDCKEEHAEFVLVRKDMLFNQLIEMALLSLGYSHSSAAQAKGLIQVGKWNPVPLSYVTDAPDATVADMLQDVYHVVTLKIQLHSGVPGVGVPGVGVPGVGVPGVGVPGVGVPGVGVPGVGVPGVGVPGVGVPGVGVPGVGVPGVGVPGVGVPGVGVPGVGVPGVGVPGVGVPGVGVPGVGVPGVGVPGVGVPGVGVPGVGVPGVGVPGVGVPGVGVPGVGVPGVGVPGVGVPGVGVPGVGVPGVGVPGVGVPGVGVPGVGVPGVGVPGVGVPGVGVPGVGVPGVGTMLPVFCVVEHYENAIEYDCKEEHAEFVLVRKDMLFNQLIEMALLSLGYSHSSAAQAKGLIQVGKWNPVPLSYVTDAPDATVADMLQDVYHVVTLKIQLHSGGREASSHHHHHH

SEQ ID NO: 91 - protein, 624 aa, Artificial Sequence
  Fusionprotein ULD-(VPGVG)80-ULD
MDPMSSSGTMLPVFCVVEHYENAIEYDCKEEHAEFVLVRKDMLFNQLIEMALLSLGYSHSSAAQAKGLIQVGKWNPVPLSYVTDAPDATVADMLQDVYHVVTLKIQLHSGVPGVGVPGVGVPGVGVPGVGVPGVGVPGVGVPGVGVPGVGVPGVGVPGVGVPGVGVPGVGVPGVGVPGVGVPGVGVPGVGVPGVGVPGVGVPGVGVPGVGVPGVGVPGVGVPGVGVPGVGVPGVGVPGVGVPGVGVPGVGVPGVGVPGVGVPGVGVPGVGVPGVGVPGVGVPGVGVPGVGVPGVGVPGVGVPGVGVPGVGVPGVGVPGVGVPGVGVPGVGVPGVGVPGVGVPGVGVPGVGVPGVGVPGVGVPGVGVPGVGVPGVGVPGVGVPGVGVPGVGVPGVGVPGVGVPGVGVPGVGVPGVGVPGVGVPGVGVPGVGVPGVGVPGVGVPGVGVPGVGVPGVGVPGVGVPGVGVPGVGVPGVGVPGVGVPGVGVPGVGVPGVGVPGVGVPGVGVPGVGTMLPVFCVVEHYENAIEYDCKEEHAEFVLVRKDMLFNQLIEMALLSLGYSHSSAAQAKGLIQVGKWNPVPLSYVTDAPDATVADMLQDVYHVVTLKIQLHSGGREASSHHHHHH

SEQ ID NO: 92 - DNA, 975 bp, Artificial Sequence
  Fusionprotein ULD-(VPGDG)20-ULD coding sequence
atggatcctatgagctcttctggtaccatgctgccggttttctgcgttgttgaacactacgaaaacgctatcgaatacgactgcaaagaagaacacgctgaatttgttctggttcgtaaagacatgctgttcaaccagctgatcgaaatggctctgctgtctctgggttactctcacagctctgctgctcaggctaaaggtctgatccaggttggtaaatggaacccggttccgctgtcttacgttaccgacgctccggacgctaccgttgctgacatgctgcaggacgtttaccacgttgttaccctgaaaatccagctgcactctggtgttccgggtgatggtgttccgggtgatggtgttccgggtgatggtgttccgggtgatggtgttccgggtgatggtgttccgggtgatggtgttccgggtgatggtgttccgggtgatggtgttccgggtgatggtgttccgggtgatggtgttccgggtgatggtgttccgggtgatggtgttccgggtgatggtgttccgggtgatggtgttccgggtgatggtgttccgggtgatggtgttccgggtgatggtgttccgggtgatggtgttccgggtgatggtgttccgggtgatggtaccatgctgccggttttctgcgttgttgaacactacgaaaacgctatcgaatacgactgcaaagaagaacacgctgaatttgttctggttcgtaaagacatgctgttcaaccagctgatcgaaatggctctgctgtctctgggttactctcacagctctgctgctcaggctaaaggtctgatccaggttggtaaatggaacccggttccgctgtcttacgttaccgacgctccggacgctaccgttgctgacatgctgcaggacgtttaccacgttgttaccctgaaaatccagctgcactctggtggaagagaagcttcatcacaccaccaccaccaccactga

SEQ ID NO: 93 - protein, 324 aa, Artificial Sequence
  Fusionprotein ULD-(VPGDG)20-ULD
MDPMSSSGTMLPVFCVVEHYENAIEYDCKEEHAEFVLVRKDMLFNQLIEMALLSLGYSHSSAAQAKGLIQVGKWNPVPLSYVTDAPDATVADMLQDVYHVVTLKIQLHSGVPGDGVPGDGVPGDGVPGDGVPGDGVPGDGVPGDGVPGDGVPGDGVPGDGVPGDGVPGDGVPGDGVPGDGVPGDGVPGDGVPGDGVPGDGVPGDGVPGDGTMLPVFCVVEHYENAIEYDCKEEHAEFVLVRKDMLFNQLIEMALLSLGYSHSSAAQAKGLIQVGKWNPVPLSYVTDAPDATVADMLQDVYHVVTLKIQLHSGGREASSHHHHHH

SEQ ID NO: 94 - DNA, 975 bp, Artificial Sequence
  Fusionprotein ULD-(VPGHG)20-ULD coding sequence
atggatcctatgagctcttctggtaccatgctgccggttttctgcgttgttgaacactacgaaaacgctatcgaatacgactgcaaagaagaacacgctgaatttgttctggttcgtaaagacatgctgttcaaccagctgatcgaaatggctctgctgtctctgggttactctcacagctctgctgctcaggctaaaggtctgatccaggttggtaaatggaacccggttccgctgtcttacgttaccgacgctccggacgctaccgttgctgacatgctgcaggacgtttaccacgttgttaccctgaaaatccagctgcactctggtgttccgggtcatggtgttccgggtcatggtgttccgggtcatggtgttccgggtcatggtgttccgggtcatggtgttccgggtcatggtgttccgggtcatggtgttccgggtcatggtgttccgggtcatggtgttccgggtcatggtgttccgggtcatggtgttccgggtcatggtgttccgggtcatggtgttccgggtcatggtgttccgggtcatggtgttccgggtcatggtgttccgggtcatggtgttccgggtcatggtgttccgggtcatggtgttccgggtcatggtaccatgctgccggttttctgcgttgttgaacactacgaaaacgctatcgaatacgactgcaaagaagaacacgctgaatttgttctggttcgtaaagacatgctgttcaaccagctgatcgaaatggctctgctgtctctgggttactctcacagctctgctgctcaggctaaaggtctgatccaggttggtaaatggaacccggttccgctgtcttacgttaccgacgctccggacgctaccgttgctgacatgctgcaggacgtttaccacgttgttaccctgaaaatccagctgcactctggtggaagagaagcttcatcacaccaccaccaccaccactga

SEQ ID NO: 95 - protein, 324 aa, Artificial Sequence
  Fusionprotein ULD-(VPGHG)20-ULD
MDPMSSSGTMLPVFCVVEHYENAIEYDCKEEHAEFVLVRKDMLFNQLIEMALLSLGYSHSSAAQAKGLIQVGKWNPVPLSYVTDAPDATVADMLQDVYHVVTLKIQLHSGVPGHGVPGHGVPGHGVPGHGVPGHGVPGHGVPGHGVPGHGVPGHGVPGHGVPGHGVPGHGVPGHGVPGHGVPGHGVPGHGVPGHGVPGHGVPGHGVPGHGTMLPVFCVVEHYENAIEYDCKEEHAEFVLVRKDMLFNQLIEMALLSLGYSHSSAAQAKGLIQVGKWNPVPLSYVTDAPDATVADMLQDVYHVVTLKIQLHSGGREASSHHHHHH

SEQ ID NO: 96 - DNA, 975 bp, Artificial Sequence
  Fusionprotein ULD-(VPGSG)20-ULD coding sequence
atggatcctatgagctcttctggtaccatgctgccggttttctgcgttgttgaacactacgaaaacgctatcgaatacgactgcaaagaagaacacgctgaatttgttctggttcgtaaagacatgctgttcaaccagctgatcgaaatggctctgctgtctctgggttactctcacagctctgctgctcaggctaaaggtctgatccaggttggtaaatggaacccggttccgctgtcttacgttaccgacgctccggacgctaccgttgctgacatgctgcaggacgtttaccacgttgttaccctgaaaatccagctgcactctggtgttccgggtagcggtgttccgggtagcggtgttccgggtagcggtgttccgggtagcggtgttccgggtagcggtgttccgggtagcggtgttccgggtagcggtgttccgggtagcggtgttccgggtagcggtgttccgggtagcggtgttccgggtagcggtgttccgggtagcggtgttccgggtagcggtgttccgggtagcggtgttccgggtagcggtgttccgggtagcggtgttccgggtagcggtgttccgggtagcggtgttccgggtagcggtgttccgggtagcggtaccatgctgccggttttctgcgttgttgaacactacgaaaacgctatcgaatacgactgcaaagaagaacacgctgaatttgttctggttcgtaaagacatgctgttcaaccagctgatcgaaatggctctgctgtctctgggttactctcacagctctgctgctcaggctaaaggtctgatccaggttggtaaatggaacccggttccgctgtcttacgttaccgacgctccggacgctaccgttgctgacatgctgcaggacgtttaccacgttgttaccctgaaaatccagctgcactctggtggaagagaagcttcatcacaccaccaccaccaccactga

SEQ ID NO: 97 - protein, 324 aa, Artificial Sequence
  Fusionprotein ULD-(VPGSG)20-ULD
MDPMSSSGTMLPVFCVVEHYENAIEYDCKEEHAEFVLVRKDMLFNQLIEMALLSLGYSHSSAAQAKGLIQVGKWNPVPLSYVTDAPDATVADMLQDVYHVVTLKIQLHSGVPGSGVPGSGVPGSGVPGSGVPGSGVPGSGVPGSGVPGSGVPGSGVPGSGVPGSGVPGSGVPGSGVPGSGVPGSGVPGSGVPGSGVPGSGVPGSGVPGSGTMLPVFCVVEHYENAIEYDCKEEHAEFVLVRKDMLFNQLIEMALLSLGYSHSSAAQAKGLIQVGKWNPVPLSYVTDAPDATVADMLQDVYHVVTLKIQLHSGGREASSHHHHHH

SEQ ID NO: 98 - DNA, 975 bp, Artificial Sequence
  Fusionprotein ULD-(VPGKG)20-ULD coding sequence
atggatcctatgagctcttctggtaccatgctgccggttttctgcgttgttgaacactacgaaaacgctatcgaatacgactgcaaagaagaacacgctgaatttgttctggttcgtaaagacatgctgttcaaccagctgatcgaaatggctctgctgtctctgggttactctcacagctctgctgctcaggctaaaggtctgatccaggttggtaaatggaacccggttccgctgtcttacgttaccgacgctccggacgctaccgttgctgacatgctgcaggacgtttaccacgttgttaccctgaaaatccagctgcactctggtgttccgggtaaaggtgttccgggtaaaggtgttccgggtaaaggtgttccgggtaaaggtgttccgggtaaaggtgttccgggtaaaggtgttccgggtaaaggtgttccgggtaaaggtgttccgggtaaaggtgttccgggtaaaggtgttccgggtaaaggtgttccgggtaaaggtgttccgggtaaaggtgttccgggtaaaggtgttccgggtaaaggtgttccgggtaaaggtgttccgggtaaaggtgttccgggtaaaggtgttccgggtaaaggtgttccgggtaaaggtaccatgctgccggttttctgcgttgttgaacactacgaaaacgctatcgaatacgactgcaaagaagaacacgctgaatttgttctggttcgtaaagacatgctgttcaaccagctgatcgaaatggctctgctgtctctgggttactctcacagctctgctgctcaggctaaaggtctgatccaggttggtaaatggaacccggttccgctgtcttacgttaccgacgctccggacgctaccgttgctgacatgctgcaggacgtttaccacgttgttaccctgaaaatccagctgcactctggtggaagagaagcttcatcacaccaccaccaccaccactga

SEQ ID NO: 99 - protein, 324 aa, Artificial Sequence
  Fusionprotein ULD-(VPGKG)20-ULD
MDPMSSSGTMLPVFCVVEHYENAIEYDCKEEHAEFVLVRKDMLFNQLIEMALLSLGYSHSSAAQAKGLIQVGKWNPVPLSYVTDAPDATVADMLQDVYHVVTLKIQLHSGVPGKGVPGKGVPGKGVPGKGVPGKGVPGKGVPGKGVPGKGVPGKGVPGKGVPGKGVPGKGVPGKGVPGKGVPGKGVPGKGVPGKGVPGKGVPGKGVPGKGTMLPVFCVVEHYENAIEYDCKEEHAEFVLVRKDMLFNQLIEMALLSLGYSHSSAAQAKGLIQVGKWNPVPLSYVTDAPDATVADMLQDVYHVVTLKIQLHSGGREASSHHHHHH

SEQ ID NO: 100 - DNA, 975 bp, Artificial Sequence; identical to SEQ ID NO: 87
  Fusionprotein ULD-(VPGRG)20-ULD coding sequence

SEQ ID NO: 101 - protein, 324 aa, Artificial Sequence; identical to SEQ ID NO: 88
  Fusionprotein ULD-(VPGRG)20-ULD

SEQ ID NO: 102 - DNA, 1035 bp, Artificial Sequence
  Fusionprotein ULD-(VPGDG-VPGSG-VPGYG)8-ULD coding sequence
atggatcctatgagctcttctggtaccatgctgccggttttctgcgttgttgaacactacgaaaacgctatcgaatacgactgcaaagaagaacacgctgaatttgttctggttcgtaaagacatgctgttcaaccagctgatcgaaatggctctgctgtctctgggttactctcacagctctgctgctcaggctaaaggtctgatccaggttggtaaatggaacccggttccgctgtcttacgttaccgacgctccggacgctaccgttgctgacatgctgcaggacgtttaccacgttgttaccctgaaaatccagctgcactctggtgttccgggtgatggtgttccgggtagcggtgttccgggttacggtgttccgggtgatggtgttccgggtagcggtgttccgggttacggtgttccgggtgatggtgttccgggtagcggtgttccgggttacggtgttccgggtgatggtgttccgggtagcggtgttccgggttacggtgttccgggtgatggtgttccgggtagcggtgttccgggttacggtgttccgggtgatggtgttccgggtagcggtgttccgggttacggtgttccgggtgatggtgttccgggtagcggtgttccgggttacggtgttccgggtgatggtgttccgggtagcggtgttccgggttacggtaccatgctgccggttttctgcgttgttgaacactacgaaaacgctatcgaatacgactgcaaagaagaacacgctgaatttgttctggttcgtaaagacatgctgttcaaccagctgatcgaaatggctctgctgtctctgggttactctcacagctctgctgctcaggctaaaggtctgatccaggttggtaaatggaacccggttccgctgtcttacgttaccgacgctccggacgctaccgttgctgacatgctgcaggacgtttaccacgttgttaccctgaaaatccagctgcactctggtggaagagaagcttcatcacaccaccaccaccaccactga

SEQ ID NO: 103 - protein, 344 aa, Artificial Sequence
  Fusionprotein ULD-(VPGDG-VPGSG-VPGYG)8-ULD
MDPMSSSGTMLPVFCVVEHYENAIEYDCKEEHAEFVLVRKDMLFNQLIEMALLSLGYSHSSAAQAKGLIQVGKWNPVPLSYVTDAPDATVADMLQDVYHVVTLKIQLHSGVPGDGVPGSGVPGYGVPGDGVPGSGVPGYGVPGDGVPGSGVPGYGVPGDGVPGSGVPGYGVPGDGVPGSGVPGYGVPGDGVPGSGVPGYGVPGDGVPGSGVPGYGVPGDGVPGSGVPGYGTMLPVFCVVEHYENAIEYDCKEEHAEFVLVRKDMLFNQLIEMALLSLGYSHSSAAQAKGLIQVGKWNPVPLSYVTDAPDATVADMLQDVYHVVTLKIQLHSGGREASSHHHHHH

SEQ ID NO: 104 - DNA, 945 bp, Artificial Sequence
  Fusionprotein ULD-(VPGVG-VPGRG-VPGYG)6-ULD coding sequence
atggatcctatgagctcttctggtaccatgctgccggttttctgcgttgttgaacactacgaaaacgctatcgaatacgactgcaaagaagaacacgctgaatttgttctggttcgtaaagacatgctgttcaaccagctgatcgaaatggctctgctgtctctgggttactctcacagctctgctgctcaggctaaaggtctgatccaggttggtaaatggaacccggttccgctgtcttacgttaccgacgctccggacgctaccgttgctgacatgctgcaggacgtttaccacgttgttaccctgaaaatccagctgcactctggtgttccgggtgttggtgttccgggtcgcggtgttccgggttacggtgttccgggtgttggtgttccgggtcgcggtgttccgggttacggtgttccgggtgttggtgttccgggtcgcggtgttccgggttacggtgttccgggtgttggtgttccgggtcgcggtgttccgggttacggtgttccgggtgttggtgttccgggtcgcggtgttccgggttacggtgttccgggtgttggtgttccgggtcgcggtgttccgggttacggtaccatgctgccggttttctgcgttgttgaacactacgaaaacgctatcgaatacgactgcaaagaagaacacgctgaatttgttctggttcgtaaagacatgctgttcaaccagctgatcgaaatggctctgctgtctctgggttactctcacagctctgctgctcaggctaaaggtctgatccaggttggtaaatggaacccggttccgctgtcttacgttaccgacgctccggacgctaccgttgctgacatgctgcaggacgtttaccacgttgttaccctgaaaatccagctgcactctggtggaagagaagcttcatcacaccaccaccaccaccactga

SEQ ID NO: 105 - protein, 314 aa, Artificial Sequence
  Fusionprotein ULD-(VPGVG-VPGRG-VPGYG)6-ULD
MDPMSSSGTMLPVFCVVEHYENAIEYDCKEEHAEFVLVRKDMLFNQLIEMALLSLGYSHSSAAQAKGLIQVGKWNPVPLSYVTDAPDATVADMLQDVYHVVTLKIQLHSGVPGVGVPGRGVPGYGVPGVGVPGRGVPGYGVPGVGVPGRGVPGYGVPGVGVPGRGVPGYGVPGVGVPGRGVPGYGVPGVGVPGRGVPGYGTMLPVFCVVEHYENAIEYDCKEEHAEFVLVRKDMLFNQLIEMALLSLGYSHSSAAQAKGLIQVGKWNPVPLSYVTDAPDATVADMLQDVYHVVTLKIQLHSGGREASSHHHHHH

SEQ ID NO: 106 - DNA, 1395 bp, Artificial Sequence
  Fusionprotein ULD-(mEGFP)-ULD, coding sequence
atggatcctatgagctcttctggtaccatgctgccggttttctgcgttgttgaacactacgaaaacgctatcgaatacgactgcaaagaagaacacgctgaatttgttctggttcgtaaagacatgctgttcaaccagctgatcgaaatggctctgctgtctctgggttactctcacagctctgctgctcaggctaaaggtctgatccaggttggtaaatggaacccggttccgctgtcttacgttaccgacgctccggacgctaccgttgctgacatgctgcaggacgtttaccacgttgttaccctgaaaatccagctgcactctggtatggtgagcaagggcgaggagctgttcaccggggtggtgcccatcctggtcgagctggacggcgacgtaaacggccacaagttcagcgtgtccggcgagggcgagggcgatgccacctacggcaagctgaccctgaagttcatctgcaccaccggcaagctgcccgtgccctggcccaccctcgtgaccaccctgacctacggcgtgcagtgcttcagccgctaccccgaccacatgaagcagcacgacttcttcaagtccgccatgcccgaaggctacgtccaggagcgcaccatcttcttcaaggacgacggcaactacaagacccgcgccgaggtgaagttcgagggcgacaccctggtgaaccgcatcgagctgaagggcatcgacttcaaggaggacggcaacatcctggggcacaagctggagtacaactacaacagccacaacgtctatatcatggccgacaagcagaagaacggcatcaaggtgaacttcaagatccgccacaacatcgaggacggcagcgtgcagctcgccgaccactaccagcagaacacccccatcggcgacggccccgtgctgctgcccgacaaccactacctgagcacccagtccaagctgagcaaagaccccaacgagaagcgcgatcacatggtcctgctggagttcgtgaccgccgccgggatcactctcggcatggacgagctgtacaagggtaccatgctgccggttttctgcgttgttgaacactacgaaaacgctatcgaatacgactgcaaagaagaacacgctgaatttgttctggttcgtaaagacatgctgttcaaccagctgatcgaaatggctctgctgtctctgggttactctcacagctctgctgctcaggctaaaggtctgatccaggttggtaaatggaacccggttccgctgtcttacgttaccgacgctccggacgctaccgttgctgacatgctgcaggacgtttaccacgttgttaccctgaaaatccagctgcactctggtggaagagaagcttcatcacaccaccaccaccaccactga

SEQ ID NO: 107 - protein, 464 aa, Artificial Sequence
  Fusionprotein ULD-(mEGFP)-ULD
MDPMSSSGTMLPVFCVVEHYENAIEYDCKEEHAEFVLVRKDMLFNQLIEMALLSLGYSHSSAAQAKGLIQVGKWNPVPLSYVTDAPDATVADMLQDVYHVVTLKIQLHSGMVSKGEELFTGVVPILVELDGDVNGHKFSVSGEGEGDATYGKLTLKFICTTGKLPVPWPTLVTTLTYGVQCFSRYPDHMKQHDFFKSAMPEGYVQERTIFFKDDGNYKTRAEVKFEGDTLVNRIELKGIDFKEDGNILGHKLEYNYNSHNVYIMADKQKNGIKVNFKIRHNIEDGSVQLADHYQQNTPIGDGPVLLPDNHYLSTQSKLSKDPNEKRDHMVLLEFVTAAGITLGMDELYKGTMLPVFCVVEHYENAIEYDCKEEHAEFVLVRKDMLFNQLIEMALLSLGYSHSSAAQAKGLIQVGKWNPVPLSYVTDAPDATVADMLQDVYHVVTLKIQLHSGGREASSHHHHHH

SEQ ID NO: 108 - DNA, 2127 bp, Artificial Sequence
  Fusion protein ULD-(mCHR-TEVrec-mEGFP)-ULD coding sequence
atggatcctatgagctcttctggtaccatgctgccggttttctgcgttgttgaacactacgaaaacgctatcgaatacgactgcaaagaagaacacgctgaatttgttctggttcgtaaagacatgctgttcaaccagctgatcgaaatggctctgctgtctctgggttactctcacagctctgctgctcaggctaaaggtctgatccaggttggtaaatggaacccggttccgctgtcttacgttaccgacgctccggacgctaccgttgctgacatgctgcaggacgtttaccacgttgttaccctgaaaatccagctgcactctggtatggtgagcaagggcgaggaggataacatggccatcatcaaggagttcatgcgcttcaaggtgcacatggagggctccgtgaacggccacgagttcgagatcgagggcgagggcgagggccgcccctacgagggcacccagaccgccaagctgaaggtgaccaagggtggccccctgcccttcgcctgggacatcctgtcccctcagttcatgtacggctccaaggcctacgtgaagcaccccgccgacatccccgactacttgaagctgtccttccccgagggcttcaagtgggagcgcgtgatgaacttcgaggacggcggcgtggtgaccgtgacccaggactcctccctgcaggacggcgagttcatctacaaggtgaagctgcgcggcaccaacttcccctccgacggccccgtaatgcagaagaagaccatgggctgggaggcctcctccgagcggatgtaccccgaggacggcgccctgaagggcgagatcaagcagaggctgaagctgaaggacggcggccactacgacgctgaggtcaagaccacctacaaggccaagaagcccgtgcagctgcccggcgcctacaacgtcaacatcaagttggacatcacctcccacaacgaggactacaccatcgtggaacagtacgaacgcgccgagggccgccactccaccggcggcatggacgagctgtacaagggtgaaaacctgtactttcagggtatggtgagcaagggcgaggagctgttcaccggggtggtgcccatcctggtcgagctggacggcgacgtaaacggccacaagttcagcgtgtccggcgagggcgagggcgatgccacctacggcaagctgaccctgaagttcatctgcaccaccggcaagctgcccgtgccctggcccaccctcgtgaccaccctgacctacggcgtgcagtgcttcagccgctaccccgaccacatgaagcagcacgacttcttcaagtccgccatgcccgaaggctacgtccaggagcgcaccatcttcttcaaggacgacggcaactacaagacccgcgccgaggtgaagttcgagggcgacaccctggtgaaccgcatcgagctgaagggcatcgacttcaaggaggacggcaacatcctggggcacaagctggagtacaactacaacagccacaacgtctatatcatggccgacaagcagaagaacggcatcaaggtgaacttcaagatccgccacaacatcgaggacggcagcgtgcagctcgccgaccactaccagcagaacacccccatcggcgacggccccgtgctgctgcccgacaaccactacctgagcacccagtccaagctgagcaaagaccccaacgagaagcgcgatcacatggtcctgctggagttcgtgaccgccgccgggatcactctcggcatggacgagctgtacaagggtaccatgctgccggttttctgcgttgttgaacactacgaaaacgctatcgaatacgactgcaaagaagaacacgctgaatttgttctggttcgtaaagacatgctgttcaaccagctgatcgaaatggctctgctgtctctgggttactctcacagctctgctgctcaggctaaaggtctgatccaggttggtaaatggaacccggttccgctgtcttacgttaccgacgctccggacgctaccgttgctgacatgctgcaggacgtttaccacgttgttaccctgaaaatccagctgcactctggtggaagagaagcttcatcacaccaccaccaccaccactga

SEQ ID NO: 109 - protein, 708 aa, Artificial Sequence
  Fusion protein ULD-(mCHR-TEVrec-mEGFP)-ULD
MDPMSSSGTMLPVFCVVEHYENAIEYDCKEEHAEFVLVRKDMLFNQLIEMALLSLGYSHSSAAQAKGLIQVGKWNPVPLSYVTDAPDATVADMLQDVYHVVTLKIQLHSGMVSKGEEDNMAIIKEFMRFKVHMEGSVNGHEFEIEGEGEGRPYEGTQTAKLKVTKGGPLPFAWDILSPQFMYGSKAYVKHPADIPDYLKLSFPEGFKWERVMNFEDGGVVTVTQDSSLQDGEFIYKVKLRGTNFPSDGPVMQKKTMGWEASSERMYPEDGALKGEIKQRLKLKDGGHYDAEVKTTYKAKKPVQLPGAYNVNIKLDITSHNEDYTIVEQYERAEGRHSTGGMDELYKGENLYFQGMVSKGEELFTGVVPILVELDGDVNGHKFSVSGEGEGDATYGKLTLKFICTTGKLPVPWPTLVTTLTYGVQCFSRYPDHMKQHDFFKSAMPEGYVQERTIFFKDDGNYKTRAEVKFEGDTLVNRIELKGIDFKEDGNILGHKLEYNYNSHNVYIMADKQKNGIKVNFKIRHNIEDGSVQLADHYQQNTPIGDGPVLLPDNHYLSTQSKLSKDPNEKRDHMVLLEFVTAAGITLGMDELYKGTMLPVFCVVEHYENAIEYDCKEEHAEFVLVRKDMLFNQLIEMALLSLGYSHSSAAQAKGLIQVGKWNPVPLSYVTDAPDATVADMLQDVYHVVTLKIQLHSGGREASSHHHHHH

SEQ ID NO: 110 - DNA, 1725 bp, Artificial Sequence
  Fusion protein ULD-(spisi10)-ULD, coding sequence
atggatcctatgagctcttctggtaccatgctgccggttttctgcgttgttgaacactacgaaaacgctatcgaatacgactgcaaagaagaacacgctgaatttgttctggttcgtaaagacatgctgttcaaccagctgatcgaaatggctctgctgtctctgggttactctcacagctctgctgctcaggctaaaggtctgatccaggttggtaaatggaacccggttccgctgtcttacgttaccgacgctccggacgctaccgttgctgacatgctgcaggacgtttaccacgttgttaccctgaaaatccagctgcactctggtcgtggtggtctgggtggtcagggtgctggtatggctgctgctgctgctatgggtggtgctggtcagggtggttacggtggtctgggttctcagggtacctctggtcgtggtggtctgggtggtcagggtgctggtatggctgctgctgctgctatgggtggtgctggtcagggtggttacggtggtctgggttctcagggtacctctggtcgtggtggtctgggtggtcagggtgctggtatggctgctgctgctgctatgggtggtgctggtcagggtggttacggtggtctgggttctcagggtacctctggtcgtggtggtctgggtggtcagggtgctggtatggctgctgctgctgctatgggtggtgctggtcagggtggttacggtggtctgggttctcagggtacctctggtcgtggtggtctgggtggtcagggtgctggtatggctgctgctgctgctatgggtggtgctggtcagggtggttacggtggtctgggttctcagggtacctctggtcgtggtggtctgggtggtcagggtgctggtatggctgctgctgctgctatgggtggtgctggtcagggtggttacggtggtctgggttctcagggtacctctggtcgtggtggtctgggtggtcagggtgctggtatggctgctgctgctgctatgggtggtgctggtcagggtggttacggtggtctgggttctcagggtacctctggtcgtggtggtctgggtggtcagggtgctggtatggctgctgctgctgctatgggtggtgctggtcagggtggttacggtggtctgggttctcagggtacctctggtcgtggtggtctgggtggtcagggtgctggtatggctgctgctgctgctatgggtggtgctggtcagggtggttacggtggtctgggttctcagggtacctctggtcgtggtggtctgggtggtcagggtgctggtatggctgctgctgctgctatgggtggtgctggtcagggtggttacggtggtctgggttctcagggtacctctggtaccatgctgccggttttctgcgttgttgaacactacgaaaacgctatcgaatacgactgcaaagaagaacacgctgaatttgttctggttcgtaaagacatgctgttcaaccagctgatcgaaatggctctgctgtctctgggttactctcacagctctgctgctcaggctaaaggtctgatccaggttggtaaatggaacccggttccgctgtcttacgttaccgacgctccggacgctaccgttgctgacatgctgcaggacgtttaccacgttgttaccctgaaaatccagctgcactctggtggaagagaagcttcatcacaccaccaccaccaccactga

SEQ ID NO: 111 - protein, 574 aa, Artificial Sequence
  Fusion protein ULD-(spisi10)-ULD
MDPMSSSGTMLPVFCVVEHYENAIEYDCKEEHAEFVLVRKDMLFNQLIEMALLSLGYSHSSAAQAKGLIQVGKWNPVPLSYVTDAPDATVADMLQDVYHVVTLKIQLHSGRGGLGGQGAGMAAAAAMGGAGQGGYGGLGSQGTSGRGGLGGQGAGMAAAAAMGGAGQGGYGGLGSQGTSGRGGLGGQGAGMAAAAAMGGAGQGGYGGLGSQGTSGRGGLGGQGAGMAAAAAMGGAGQGGYGGLGSQGTSGRGGLGGQGAGMAAAAAMGGAGQGGYGGLGSQGTSGRGGLGGQGAGMAAAAAMGGAGQGGYGGLGSQGTSGRGGLGGQGAGMAAAAAMGGAGQGGYGGLGSQGTSGRGGLGGQGAGMAAAAAMGGAGQGGYGGLGSQGTSGRGGLGGQGAGMAAAAAMGGAGQGGYGGLGSQGTSGRGGLGGQGAGMAAAAAMGGAGQGGYGGLGSQGTSGTMLPVFCVVEHYENAIEYDCKEEHAEFVLVRKDMLFNQLIEMALLSLGYSHSSAAQAKGLIQVGKWNPVPLSYVTDAPDATVADMLQDVYHVVTLKIQLHSGGREASSHHHHHH

SEQ ID NO: 112 - DNA, 1125 bp, Artificial Sequence
  Fusion protein ULD-(resi10)-ULD, cosing sequence
atggatcctatgagctcttctggtaccatgctgccggttttctgcgttgttgaacactacgaaaacgctatcgaatacgactgcaaagaagaacacgctgaatttgttctggttcgtaaagacatgctgttcaaccagctgatcgaaatggctctgctgtctctgggttactctcacagctctgctgctcaggctaaaggtctgatccaggttggtaaatggaacccggttccgctgtcttacgttaccgacgctccggacgctaccgttgctgacatgctgcaggacgtttaccacgttgttaccctgaaaatccagctgcactctggtggtcgaccttctgattcttacggtgctcctggtggtggtaatggtggtcgaccttctgattcttacggtgctcctggtggtggtaatggtggtcgaccttctgattcttacggtgctcctggtggtggtaatggtggtcgaccttctgattcttacggtgctcctggtggtggtaatggtggtcgaccttctgattcttacggtgctcctggtggtggtaatggtggtcgaccttctgattcttacggtgctcctggtggtggtaatggtggtcgaccttctgattcttacggtgctcctggtggtggtaatggtggtcgaccttctgattcttacggtgctcctggtggtggtaatggtggtcgaccttctgattcttacggtgctcctggtggtggtaatggtggtcgaccttctgattcttacggtgctcctggtggtggtaatggtaccatgctgccggttttctgcgttgttgaacactacgaaaacgctatcgaatacgactgcaaagaagaacacgctgaatttgttctggttcgtaaagacatgctgttcaaccagctgatcgaaatggctctgctgtctctgggttactctcacagctctgctgctcaggctaaaggtctgatccaggttggtaaatggaacccggttccgctgtcttacgttaccgacgctccggacgctaccgttgctgacatgctgcaggacgtttaccacgttgttaccctgaaaatccagctgcactctggtggaagagaagcttcatcacaccaccaccaccaccactga

SEQ ID NO: 113 - protein, 374 aa, Artificial Sequence
  Fusion protein ULD-(resi10)-ULD
MDPMSSSGTMLPVFCVVEHYENAIEYDCKEEHAEFVLVRKDMLFNQLIEMALLSLGYSHSSAAQAKGLIQVGKWNPVPLSYVTDAPDATVADMLQDVYHVVTLKIQLHSGGRPSDSYGAPGGGNGGRPSDSYGAPGGGNGGRPSDSYGAPGGGNGGRPSDSYGAPGGGNGGRPSDSYGAPGGGNGGRPSDSYGAPGGGNGGRPSDSYGAPGGGNGGRPSDSYGAPGGGNGGRPSDSYGAPGGGNGGRPSDSYGAPGGGNGTMLPVFCVVEHYENAIEYDCKEEHAEFVLVRKDMLFNQLIEMALLSLGYSHSSAAQAKGLIQVGKWNPVPLSYVTDAPDATVADMLQDVYHVVTLKIQLHSGGREASSHHHHHH

SEQ ID NO: 114 - DNA, 2433 bp, Artificial Sequence
  Fusion protein ULD-(hsa)-ULD, hsa = human serum albumin, coding sequence
atggatcctatgagctcttctggtaccatgctgccggttttctgcgttgttgaacactacgaaaacgctatcgaatacgactgcaaagaagaacacgctgaatttgttctggttcgtaaagacatgctgttcaaccagctgatcgaaatggctctgctgtctctgggttactctcacagctctgctgctcaggctaaaggtctgatccaggttggtaaatggaacccggttccgctgtcttacgttaccgacgctccggacgctaccgttgctgacatgctgcaggacgtttaccacgttgttaccctgaaaatccagctgcactctggtgacgctcacaaatctgaagttgctcaccgtttcaaagacctgggtgaagaaaacttcaaagctctggttctgatcgctttcgctcagtacctgcagcagtgcccgttcgaagaccacgttaaactggttaacgaagttaccgaatttgctaaaacctgcgttgctgacgaatctgctgaaaactgcgacaaatctctgcacaccctgttcggtgacaaactgtgtaccgttgctaccctgcgtgaaacctacggtgaaatggctgactgctgcgctaaacaggaaccggaacgtaacgaatgcttcctgcagcacaaagacgacaacccgaacctgccgcgtctggttcgtccggaagttgacgttatgtgtaccgctttccacgacaacgaagaaaccttcctgaaaaaatacctgtacgaaatcgctcgtcgtcacccgtacttctacgctccggaactgctgttcttcgctaaacgttacaaagctgctttcaccgaatgctgccaggctgctgacaaagctgcttgcctgctgccgaaactggacgaactgcgtgacgaaggtaaagcgtcttctgctaaacagcgtctgaaatgcgcttctctgcagaaattcggtgaacgtgctttcaaagcgtgggctgttgctcgtctgtctcagcgtttcccgaaagctgaatttgctgaagtttctaaactggttaccgacctgaccaaagttcacaccgaatgctgccacggtgacctgctggaatgcgctgacgaccgtgctgacctggctaaatacatctgcgaaaaccaggactctatctcgtctaaactgaaagaatgctgcgaaaaaccgctgctggaaaaatctcactgcatcgctgaagttgaaaacgacgaaatgccggctgacctgccgtctctggctgctgacttcgttgaatctaaagacgtttgcaaaaactacgctgaagctaaagacgttttcctgggtatgttcctgtacgaatacgctcgtcgtcacccggactactctgttgttctgctgctgcgtctggctaaaacctacgaaaccaccctggaaaaatgctgcgctgctgctgacccgcacgaatgctacgctaaagttttcgacgagttcaaaccgctggttgaagaaccgcagaacctgatcaaacagaactgcgaactgttcgaacagctgggtgaatacaaattccagaacgctctgctggttcgttacaccaaaaaagttccgcaggtttctaccccgaccctggttgaagtttctcgtaacctgggtaaagttggttctaaatgctgcaaacacccggaagctaaacgtatgccgtgcgctgaagactacctgtctgttgttctgaaccagctgtgcgttctgcacgaaaaaaccccggtttctgaccgtgttaccaaatgctgcaccgaatctctggttaaccgtcgtccgtgcttctctgctctggaagttgacgaaacctacgttccgaaagagttcaacgctgaaaccttcaccttccacgctgacatctgcaccctgtctgaaaaagaacgtcagatcaaaaaacagaccgctctggttgaactggttaaacacaaaccgaaagctaccaaagaacagctgaaagctgttatggacgacttcgctgctttcgttgaaaaatgctgcaaagctgacgacaaagaaacctgcttcgctgaagaaggtaaaaaactggttgctgcttctcaggctgctctgggtctgggtaccatgctgccggttttctgcgttgttgaacactacgaaaacgctatcgaatacgactgcaaagaagaacacgctgaatttgttctggttcgtaaagacatgctgttcaaccagctgatcgaaatggctctgctgtctctgggttactctcacagctctgctgctcaggctaaaggtctgatccaggttggtaaatggaacccggttccgctgtcttacgttaccgacgctccggacgctaccgttgctgacatgctgcaggacgtttaccacgttgttaccctgaaaatccagctgcactctggtggaagagaagcttcatcacaccaccaccaccaccactga

SEQ ID NO: 115 - protein, 810 aa, Artificial Sequence
  Fusion protein ULD-(hsa)-ULD, hsa = human serum albumin
MDPMSSSGTMLPVFCVVEHYENAIEYDCKEEHAEFVLVRKDMLFNQLIEMALLSLGYSHSSAAQAKGLIQVGKWNPVPLSYVTDAPDATVADMLQDVYHVVTLKIQLHSGDAHKSEVAHRFKDLGEENFKALVLIAFAQYLQQCPFEDHVKLVNEVTEFAKTCVADESAENCDKSLHTLFGDKLCTVATLRETYGEMADCCAKQEPERNECFLQHKDDNPNLPRLVRPEVDVMCTAFHDNEETFLKKYLYEIARRHPYFYAPELLFFAKRYKAAFTECCQAADKAACLLPKLDELRDEGKASSAKQRLKCASLQKFGERAFKAWAVARLSQRFPKAEFAEVSKLVTDLTKVHTECCHGDLLECADDRADLAKYICENQDSISSKLKECCEKPLLEKSHCIAEVENDEMPADLPSLAADFVESKDVCKNYAEAKDVFLGMFLYEYARRHPDYSVVLLLRLAKTYETTLEKCCAAADPHECYAKVFDEFKPLVEEPQNLIKQNCELFEQLGEYKFQNALLVRYTKKVPQVSTPTLVEVSRNLGKVGSKCCKHPEAKRMPCAEDYLSVVLNQLCVLHEKTPVSDRVTKCCTESLVNRRPCFSALEVDETYVPKEFNAETFTFHADICTLSEKERQIKKQTALVELVKHKPKATKEQLKAVMDDFAAFVEKCCKADDKETCFAEEGKKLVAASQAALGLGTMLPVFCVVEHYENAIEYDCKEEHAEFVLVRKDMLFNQLIEMALLSLGYSHSSAAQAKGLIQVGKWNPVPLSYVTDAPDATVADMLQDVYHVVTLKIQLHSGGREASSHHHHHH

SEQ ID NO: 116 - DNA, 369 bp, Artificial Sequence
  N-terminal domain of human SATB1 with methionin and fusion peptide linker sequence (N-terminal, DPMSSS), and fusion peptide linker sequence and His-tag (C-terminal, GGREASS and His6)
atggatcctatgagctcttctggtaccatgctgccggttttctgcgttgttgaacactacgaaaacgctatcgaatacgactgcaaagaagaacacgctgaatttgttctggttcgtaaagacatgctgttcaaccagctgatcgaaatggctctgctgtctctgggttactctcacagctctgctgctcaggctaaaggtctgatccaggttggtaaatggaacccggttccgctgtcttacgttaccgacgctccggacgctaccgttgctgacatgctgcaggacgtttaccacgttgttaccctgaaaatccagctgcactctggtggaagagaagcttcatcacaccaccaccaccaccactga

SEQ ID NO: 117 - protein, 122 aa, Artificial Sequence
  N-terminal domain of human SATB1 with methionin and fusion peptide linker sequence (N-terminal, DPMSSS), and fusion peptide linker sequence and His-tag (C-terminal, GGREASS and His6)
MDPMSSSGTMLPVFCVVEHYENAIEYDCKEEHAEFVLVRKDMLFNQLIEMALLSLGYSHSSAAQAKGLIQVGKWNPVPLSYVTDAPDATVADMLQDVYHVVTLKIQLHSGGREASSHHHHHH